European Patent Application EP 4 046 655 A9, published April 12, 2023. Title: Antibodies specifically binding PD-1 and their uses. Applicant: DeAngelis, Nikki A Powers, Gordon Sabins, Nina  Chi Santulli-Marotto, Sandra Verona, Raluca Wiehagen, Karla R. Application To Be Assigned. The sequence listing filed with the application follows.

SEQUENCE LISTING (312 sequences)

SEQ ID NO: 1 - protein, 268 aa, Homo sapiens
PGWFLDSPDRPWNPPTFSPALLVVTEGDNATFTCSFSNTSESFVLNWYRMSPSNQTDKLAAFPEDRSQPGQDCRFRVTQLPNGRDFHMSVVRARRNDSGTYLCGAISLAPKAQIKESLRAELRVTERRAEVPTAHPSPSPRPAGQFQTLVVGVVGGLLGSLVLLVWVLAVICSRAARGTIGARRTGQPLKEDPSAVPVFSVDYGELDFQWREKTPEPPVPCVPEQTEYATIVFPSGMGTSSPARRGSADGPRSAQPLRPEDGHCSWPL

SEQ ID NO: 2 - protein, 149 aa, Homo sapiens
PGWFLDSPDRPWNPPTFSPALLVVTEGDNATFTCSFSNTSESFVLNWYRMSPSNQTDKLAAFPEDRSQPGQDCRFRVTQLPNGRDFHMSVVRARRNDSGTYLCGAISLAPKAQIKESLRAELRVTERRAEVPTAHPSPSPRPAGQFQTL

SEQ ID NO: 3 - protein, 268 aa, Macaca fascicularis
PGWFLESPDRPWNAPTFSPALLLVTEGDNATFTCSFSNASESFVLNWYRMSPSNQTDKLAAFPEDRSQPGQDCRFRVTRLPNGRDFHMSVVRARRNDSGTYLCGAISLAPKAQIKESLRAELRVTERRAEVPTAHPSPSPRPAGQFQALVVGVVGGLLGSLVLLVWVLAVICSRAAQGTIEARRTGQPLKEDPSAVPVFSVDYGELDFQWREKTPEPPAPCVPEQTEYATIVFPSGLGTSSPARRGSADGPRSPRPLRPEDGHCSWPL

SEQ ID NO: 4 - protein, 149 aa, Macaca fascicularis
PGWFLESPDRPWNAPTFSPALLLVTEGDNATFTCSFSNASESFVLNWYRMSPSNQTDKLAAFPEDRSQPGQDCRFRVTRLPNGRDFHMSVVRARRNDSGTYLCGAISLAPKAQIKESLRAELRVTERRAEVPTAHPSPSPRPAGQFQAL

SEQ ID NO: 5 - protein, 220 aa, Homo sapiens
FTVTVPKDLYVVEYGSNMTIECKFPVEKQLDLAALIVYWEMEDKNIIQFVHGEEDLKVQHSSYRQRARLLKDQLSLGNAALQITDVKLQDAGVYRCMISYGGADYKRITVKVNAPYNKINQRILVVDPVTSEHELTCQAEGYPKAEVIWTSSDHQVLSGKTTTTNSKREEKLFNVTSTLRINTTTNEIFYCTFRRLDPEENHTAELVIPELPLAHPPNER

SEQ ID NO: 6 - protein, 221 aa, Homo sapiens [sequence omitted]

SEQ ID NO: 7 - protein, 222 aa, Macaca fascicularis
AFTVTVPKDLYVVEYGSNMTIECKFPVEKQLDLTSLIVYWEMEDKNIIQFVHGEEDLKVQHSNYRQRAQLLKDQLSLGNAALRITDVKLQDAGVYRCMISYGGADYKRITVKVNAPYNKINQRILVVDPVTSEHELTCQAEGYPKAEVIWTSSDHQVLSGKTTTTNSKREEKLLNVTSTLRINTTANEIFYCIFRRLDPEENHTAELVIPELPLALPPNERT

SEQ ID NO: 8 - protein, 201 aa, Homo sapiens
LFTVTVPKELYIIEHGSNVTLECNFDTGSHVNLGAITASLQKVENDTSPHRERATLLEEQLPLGKASFHIPQVQVRDEGQYQCIIIYGVAWDYKYLTLKVKASYRKINTHILKVPETDEVELTCQATGYPLAEVSWPNVSVPANTSHSRTPEGLYQVTSVLRLKPPPGRNFSCVFWNTHVRELTLASIDLQSQMEPRTHPT

SEQ ID NO: 9 - protein, 143 aa, Mus musculus
LEVPNGPWRSLTFYPAWLTVSEGANATFTCSLSNWSEDLMLNWNRLSPSNQTEKQAAFCNGLSQPVQDARFQIIQLPNRHDFHMNILDTRRNDSGIYLCGAISLHPKAKIEESPGAELVVTERILETSTRYPSPSPKPEGRFQ

SEQ ID NO: 10 - protein, 5 aa, Artificial sequence
  PD-1 antibody HCDR1
SYAIS

SEQ ID NO: 11 - protein, 5 aa, Artificial sequence
  PD-1 antibody HCDR1
DYVIS

SEQ ID NO: 12 - protein, 5 aa, Artificial sequence
  PD-1 antibody HCDR1
SYVIH

SEQ ID NO: 13 - protein, 17 aa, Artificial sequence
  PD-1 antibody HCDR2
GIIPIFGTANYAQKFQG

SEQ ID NO: 14 - protein, 17 aa, Artificial sequence
  PD-1 antibody HCDR2
GIIPIFDTANYAQKFQG

SEQ ID NO: 15 - protein, 17 aa, Artificial sequence
  PD-1 antibody HCDR2
GIIPIYGTANYAQKFQG

SEQ ID NO: 16 - protein, 14 aa, Artificial sequence
  PD-1 antibody HCDR3
PGLAAAYDTGNLDY

SEQ ID NO: 17 - protein, 14 aa, Artificial sequence
  PD-1 antibody HCDR3
PGLAAAYDTGSLDY

SEQ ID NO: 18 - protein, 11 aa, Artificial sequence
  PD-1 antibody HCDR3
GTLDRTGHLDY

SEQ ID NO: 19 - protein, 11 aa, Artificial sequence
  PD-1 antibody HCDR3
GYVRATGMLDY

SEQ ID NO: 20 - protein, 11 aa, Artificial sequence
  PD-1 antibody LCDR1
RASQSVSSYLA

SEQ ID NO: 21 - protein, 11 aa, Artificial sequence
  PD-1 antibody LCDR1
RASQSVRNYLA

SEQ ID NO: 22 - protein, 11 aa, Artificial sequence
  PD-1 antibody LCDR1
RASQSVDSYLA

SEQ ID NO: 23 - protein, 11 aa, Artificial sequence
  PD-1 antibody LCDR1
RASQSVRSYLA

SEQ ID NO: 24 - protein, 11 aa, Artificial sequence
  PD-1 antibody LCDR1
RASQSVSNYLA

SEQ ID NO: 25 - protein, 11 aa, Artificial sequence
  PD-1 antibody LCDR1
RASQSVDNYLA

SEQ ID NO: 26 - protein, 7 aa, Artificial sequence
  PD-1 antibody LCDR2
DASNRAT

SEQ ID NO: 27 - protein, 7 aa, Artificial sequence
  PD-1 antibody LCDR2
DASDRAT

SEQ ID NO: 28 - protein, 7 aa, Artificial sequence
  PD-1 antibody LCDR2
DASYRAT

SEQ ID NO: 29 - protein, 7 aa, Artificial sequence
  PD-1 antibody LCDR2
DASSRAT

SEQ ID NO: 30 - protein, 7 aa, Artificial sequence
  PD-1 antibody LCDR2
DASTRAT

SEQ ID NO: 31 - protein, 9 aa, Artificial sequence
  PD-1 antibody LCDR3
QQRSNWPLT

SEQ ID NO: 32 - protein, 9 aa, Artificial sequence
  PD-1 antibody LCDR3
QQRNYWPLT

SEQ ID NO: 33 - protein, 9 aa, Artificial sequence
  PD-1 antibody LCDR3
QQRGNWPLT

SEQ ID NO: 34 - protein, 9 aa, Artificial sequence
  PD-1 antibody LCDR3
QQREYWPLT

SEQ ID NO: 35 - protein, 9 aa, Artificial sequence
  PD-1 antibody LCDR3
QQRDYWPLT

SEQ ID NO: 36 - protein, 9 aa, Artificial sequence
  PD-1 antibody LCDR3
QQRGYWPLT

SEQ ID NO: 37 - protein, 9 aa, Artificial sequence
  PD-1 antibody LCDR3
QQRWNWPLT

SEQ ID NO: 38 - protein, 9 aa, Artificial sequence
  PD-1 antibody LCDR3
QQRAYWPLT

SEQ ID NO: 39 - protein, 9 aa, Artificial sequence
  PD-1 antibody LCDR3
QQRAEWPLT

SEQ ID NO: 40 - protein, 9 aa, Artificial sequence
  PD-1 antibody LCDR3
QQRSAWPLT

SEQ ID NO: 41 - protein, 123 aa, Artificial sequence
  PD1H24
QVQLVQSGAEVKKPGSSVKVSCKASGGTFSSYAISWVRQAPGQGLEWMGGIIPIFGTANYAQKFQGRVTITADESTSTAYMELSSLRSEDTAVYYCARPGLAAAYDTGNLDYWGQGTLVTVSS

SEQ ID NO: 42 - protein, 123 aa, Artificial sequence
  PD1H131
QVQLVQSGAEVKKPGSSVKVSCKASGGTFSSYAISWVRQAPGQGLEWMGGIIPIFDTANYAQKFQGRVTITADESTSTAYMELSSLRSEDTAVYYCARPGLAAAYDTGNLDYWGQGTLVTVSS

SEQ ID NO: 43 - protein, 123 aa, Artificial sequence
  PD1H3
QVQLVQSGAEVKKPGSSVKVSCKASGGTFSSYAISWVRQAPGQGLEWMGGIIPIFGTANYAQKFQGRVTITADESTSTAYMELSSLRSEDTAVYYCARPGLAAAYDTGSLDYWGQGTLVTVSS

SEQ ID NO: 44 - protein, 120 aa, Artificial sequence
  PD1H108
QVQLVQSGAEVKKPGSSVKVSCKASGGTFSSYAISWVRQAPGQGLEWMGGIIPIFGTANYAQKFQGRVTITADESTSTAYMELSSLRSEDTAVYYCARGTLDRTGHLDYWGQGTLVTVSS

SEQ ID NO: 45 - protein, 120 aa, Artificial sequence
  PD1H164
QVQLVQSGAEVKKPGSSVKVSCKASGGTFSDYVISWVRQAPGQGLEWMGGIIPIYGTANYAQKFQGRVTITADESTSTAYMELSSLRSEDTAVYYCARGTLDRTGHLDYWGQGTLVTVSS

SEQ ID NO: 46 - protein, 120 aa, Artificial sequence
  PD1H107
QVQLVQSGAEVKKPGSSVKVSCKASGGTFSSYAISWVRQAPGQGLEWMGGIIPIFGTANYAQKFQGRVTITADESTSTAYMELSSLRSEDTAVYYCARGYVRATGMLDYWGQGTLVTVSS

SEQ ID NO: 47 - protein, 120 aa, Artificial sequence
  PD1H163
QVQLVQSGAEVKKPGSSVKVSCKASGGTFKSYVIHWVRQAPGQGLEWMGGIIPIFGTANYAQKFQGRVTITADESTSTAYMELSSLRSEDTAVYYCARGYVRATGMLDYWGQGTLVTVSS

SEQ ID NO: 48 - protein, 123 aa, Artificial sequence
  PD1H170
QVQLVQSGAEVKKPGSSVKVSCKASGGTFSSYAISWVRQAPGQGLEWMGGIIPIFDTANYAQKFQGRVTITADESTSTAYMELSSLRSEDTAVYYCARPGLAAAYDTGSLDYWGQGTLVTVSS

SEQ ID NO: 49 - protein, 107 aa, Artificial sequence
  PH9L3
EIVLTQSPATLSLSPGERATLSCRASQSVSSYLAWYQQKPGQAPRLLIYDASNRATGIPARFSGSGSGTDFTLTISSLEPEDFAVYYCQQRSNWPLTFGQGTKVEIK

SEQ ID NO: 50 - protein, 107 aa, Artificial sequence
  PD1L128
EIVLTQSPATLSLSPGERATLSCRASQSVRNYLAWYQQKPGQAPRLLIHDASNRATGIPARFSGSGSGTDFTLTISSLEPEDFAVYYCQQRNYWPLTFGQGTKVEIK

SEQ ID NO: 51 - protein, 107 aa, Artificial sequence
  PD1L101
EIVLTQSPATLSLSPGERATLSCRASQSVDSYLAWYQQKPGQAPRLLIKDASDRATGIPARFSGSGSGTDFTLTISSLEPEDFAVYYCQQRGNWPLTFGQGTKVEIK

SEQ ID NO: 52 - protein, 107 aa, Artificial sequence
  PD1L67
EIVLTQSPATLSLSPGERATLSCRASQSVDSYLAWYQQKPGQAPRLLIYDASNRATGIPARFSGSGSGTDFTLTISSLEPEDFAVYYCQQREYWPLTFGQGTKVEIK

SEQ ID NO: 53 - protein, 107 aa, Artificial sequence
  PD1L71
EIVLTQSPATLSLSPGERATLSCRASQSVRSYLAWYQQKPGQAPRLLIYDASYRATGIPARFSGSGSGTDFTLTISSLEPEDFAVYYCQQRDYWPLTFGQGTKVEIK

SEQ ID NO: 54 - protein, 107 aa, Artificial sequence
  PD1L109
EIVLTQSPATLSLSPGERATLSCRASQSVSSYLAWYQQKPGQAPRLLIKDASNRATGIPARFSGSGSGTDFTLTISSLEPEDFAVYYCQQRGYWPLTFGQGTKVEIK

SEQ ID NO: 55 - protein, 107 aa, Artificial sequence
  PD1L132
EIVLTQSPATLSLSPGERATLSCRASQSVRNYLAWYQQKPGQAPRLLIYDASDRATGIPARFSGSGSGTDFTLTISSLEPEDFAVYYCQQRWNWPLTFGQGTKVEIK

SEQ ID NO: 56 - protein, 107 aa, Artificial sequence
  PD1L148
EIVLTQSPATLSLSPGERATLSCRASQSVRSYLAWYQQKPGQAPRLLIYDASNRATGIPARFSGSGSGTDFTLTISSLEPEDFAVYYCQQRNYWPLTFGQGTKVEIK

SEQ ID NO: 57 - protein, 107 aa, Artificial sequence
  PD1L133
EIVLTQSPATLSLSPGERATLSCRASQSVDSYLAWYQQKPGQAPRLLIHDASNRATGIPARFSGSGSGTDFTLTISSLEPEDFAVYYCQQRNYWPLTFGQGTKVEIK

SEQ ID NO: 58 - protein, 107 aa, Artificial sequence
  PD1L185
EIVLTQSPATLSLSPGERATLSCRASQSVSNYLAWYQQKPGQAPRLLIYDASNRATGIPARFSGSGSGTDFTLTISSLEPEDFAVYYCQQRAYWPLTFGQGTKVEIK

SEQ ID NO: 59 - protein, 107 aa, Artificial sequence
  PD1L187
EIVLTQSPATLSLSPGERATLSCRASQSVSSYLAWYQQKPGQAPRLLIEDASSRATGIPARFSGSGSGTDFTLTISSLEPEDFAVYYCQQRAEWPLTFGQGTKVEIK

SEQ ID NO: 60 - protein, 107 aa, Artificial sequence
  PD1L86
EIVLTQSPATLSLSPGERATLSCRASQSVSSYLAWYQQKPGQAPRLLIHDASTRATGIPARFSGSGSGTDFTLTISSLEPEDFAVYYCQQRNYWPLTFGQGTKVEIK

SEQ ID NO: 61 - protein, 107 aa, Artificial sequence
  PD1L168
EIVLTQSPATLSLSPGERATLSCRASQSVDNYLAWYQQKPGQAPRLLIHDASNRATGIPARFSGSGSGTDFTLTISSLEPEDFAVYYCQQRSAWPLTFGQGTKVEIK

SEQ ID NO: 62 - protein, 107 aa, Artificial sequence
  PD1L190
EIVLTQSPATLSLSPGERATLSCRASQSVSNYLAWYQQKPGQAPRLLIYDASNRATGIPARFSGSGSGTDFTLTISSLEPEDFAVYYCQQRNYWPLTFGQGTKVEIK

SEQ ID NO: 63 - protein, 117 aa, Artificial sequence
  PD1H130
EVQLVESGGGLVQPGGSLRLSCAASGFAFSRYDMSWIRLAPGKGLESVAYISGGGANTYYLDNVKGRFTISRDNAKNSLYLQMNSLRAEDTAVYYCASPYLSYFDVWGQGTLVTVSS

SEQ ID NO: 64 - protein, 117 aa, Artificial sequence
  PD1H129
EVQLVESGGGLVQPGGSLRLSCAASGFAFSRYDMSWVRQAPGKGLESVAYISGGGANTYYLDNVKGRFTISRDNAKNSLYLQMNSLRAEDTAVYYCASPYLSYFDVWGQGTLVTVSS

SEQ ID NO: 65 - protein, 107 aa, Artificial sequence
  PD1L62
EIVMTQSPATLSVSPGERATLSCRASQSLSDYLHWYQQKPGQAPRLLIKSASQSISGIPARFSGSGSGTEFTLTISSLQSEDFAVYYCQNGHSFPYTFGQGTKLEIK

SEQ ID NO: 66 - protein, 5 aa, Artificial sequence
  PD1 antibody HCDR1
RYDMS

SEQ ID NO: 67 - protein, 17 aa, Artificial sequence
  PD1 antibody HCDR2
YISGGGANTYYLDNVKG

SEQ ID NO: 68 - protein, 8 aa, Artificial sequence
  PD1 antibody HCDR3
PYLSYFDV

SEQ ID NO: 69 - protein, 11 aa, Artificial sequence
  PD1 antibody LCDR1
RASQSLSDYLH

SEQ ID NO: 70 - protein, 7 aa, Artificial sequence
  PD1 antibody LCDR2
SASQSIS

SEQ ID NO: 71 - protein, 9 aa, Artificial sequence
  PD1 antibody LCDR3
QNGHSFPYT

SEQ ID NO: 72 - protein, 450 aa, Artificial sequence
  PD1B244 HC
QVQLVQSGAEVKKPGSSVKVSCKASGGTFSSYAISWVRQAPGQGLEWMGGIIPIFDTANYAQKFQGRVTITADESTSTAYMELSSLRSEDTAVYYCARPGLAAAYDTGSLDYWGQGTLVTVSSASTKGPSVFPLAPCSRSTSESTAALGCLVKDYFPEPVTVSWNSGALTSGVHTFPAVLQSSGLYSLSSVVTVPSSSLGTKTYTCNVDHKPSNTKVDKRVESKYGPPCPPCPAPEFLGGPSVFLFPPKPKDTLMISRTPEVTCVVVDVSQEDPEVQFNWYVDGVEVHNAKTKPREEQFNSTYRVVSVLTVLHQDWLNGKEYKCKVSNKGLPSSIEKTISKAKGQPREPQVYTLPPSQEEMTKNQVSLTCLVKGFYPSDIAVEWESNGQPENNYKTTPPVLDSDGSFFLYSRLTVDKSRWQEGNVFSCSVMHEALHNHYTQKSLSLSLGK

SEQ ID NO: 73 - protein, 214 aa, Artificial sequence
  PD1B244 LC
EIVLTQSPATLSLSPGERATLSCRASQSVRSYLAWYQQKPGQAPRLLIYDASNRATGIPARFSGSGSGTDFTLTISSLEPEDFAVYYCQQRNYWPLTFGQGTKVEIKRTVAAPSVFIFPPSDEQLKSGTASVVCLLNNFYPREAKVQWKVDNALQSGNSQESVTEQDSKDSTYSLSSTLTLSKADYEKHKVYACEVTHQGLSSPVTKSFNRGEC

SEQ ID NO: 74 - protein, 444 aa, Artificial sequence
  PD1B243 HC
EVQLVESGGGLVQPGGSLRLSCAASGFAFSRYDMSWVRQAPGKGLESVAYISGGGANTYYLDNVKGRFTISRDNAKNSLYLQMNSLRAEDTAVYYCASPYLSYFDVWGQGTLVTVSSASTKGPSVFPLAPCSRSTSESTAALGCLVKDYFPEPVTVSWNSGALTSGVHTFPAVLQSSGLYSLSSVVTVPSSSLGTKTYTCNVDHKPSNTKVDKRVESKYGPPCPPCPAPEFLGGPSVFLFPPKPKDTLMISRTPEVTCVVVDVSQEDPEVQFNWYVDGVEVHNAKTKPREEQFNSTYRVVSVLTVLHQDWLNGKEYKCKVSNKGLPSSIEKTISKAKGQPREPQVYTLPPSQEEMTKNQVSLTCLVKGFYPSDIAVEWESNGQPENNYKTTPPVLDSDGSFFLYSRLTVDKSRWQEGNVFSCSVMHEALHNHYTQKSLSLSLGK

SEQ ID NO: 75 - protein, 214 aa, Artificial sequence
  PD1B243 LC
EIVMTQSPATLSVSPGERATLSCRASQSLSDYLHWYQQKPGQAPRLLIKSASQSISGIPARFSGSGSGTEFTLTISSLQSEDFAVYYCQNGHSFPYTFGQGTKLEIKRTVAAPSVFIFPPSDEQLKSGTASVVCLLNNFYPREAKVQWKVDNALQSGNSQESVTEQDSKDSTYSLSSTLTLSKADYEKHKVYACEVTHQGLSSPVTKSFNRGEC

SEQ ID NO: 76 - protein, 447 aa, Artificial sequence
  PD1B245 HC
QVQLVQSGAEVKKPGSSVKVSCKASGGTFSDYVISWVRQAPGQGLEWMGGIIPIYGTANYAQKFQGRVTITADESTSTAYMELSSLRSEDTAVYYCARGTLDRTGHLDYWGQGTLVTVSSASTKGPSVFPLAPCSRSTSESTAALGCLVKDYFPEPVTVSWNSGALTSGVHTFPAVLQSSGLYSLSSVVTVPSSSLGTKTYTCNVDHKPSNTKVDKRVESKYGPPCPPCPAPEFLGGPSVFLFPPKPKDTLMISRTPEVTCVVVDVSQEDPEVQFNWYVDGVEVHNAKTKPREEQFNSTYRVVSVLTVLHQDWLNGKEYKCKVSNKGLPSSIEKTISKAKGQPREPQVYTLPPSQEEMTKNQVSLTCLVKGFYPSDIAVEWESNGQPENNYKTTPPVLDSDGSFFLYSRLTVDKSRWQEGNVFSCSVMHEALHNHYTQKSLSLSLGK

SEQ ID NO: 77 - protein, 214 aa, Artificial sequence
  PD1B245 LC
EIVLTQSPATLSLSPGERATLSCRASQSVSSYLAWYQQKPGQAPRLLIHDASTRATGIPARFSGSGSGTDFTLTISSLEPEDFAVYYCQQRNYWPLTFGQGTKVEIKRTVAAPSVFIFPPSDEQLKSGTASVVCLLNNFYPREAKVQWKVDNALQSGNSQESVTEQDSKDSTYSLSSTLTLSKADYEKHKVYACEVTHQGLSSPVTKSFNRGEC

SEQ ID NO: 78 - protein, 443 aa, Artificial sequence
  TIM3 antibody heavy chain
EVQLLESGGGLVQPGGSLRLSCAASGFTFSSYAMSWVRQAPGKGLEWVSAISGSGGSTYYADSVKGRFTISRDNSKNTLYLQMNSLRAEDTAVYYCAKSPYAPLDYWGQGTLVTVSSASTKGPSVFPLAPCSRSTSESTAALGCLVKDYFPEPVTVSWNSGALTSGVHTFPAVLQSSGLYSLSSVVTVPSSNFGTQTYTCNVDHKPSNTKVDKTVERKCCVECPPCPAPPAAASSVFLFPPKPKDTLMISRTPEVTCVVVDVSAEDPEVQFNWYVDGVEVHNAKTKPREEQFNSTFRVVSVLTVLHQDWLNGKEYKCKVSNKGLPSSIEKTISKTKGQPREPQVYTLPPSREEMTKNQVSLTCLVKGFYPSDIAVEWESNGQPENNYKTTPPMLDSDGSFFLYSKLTVDKSRWQQGNVFSCSVMHEALHNHYTQKSLSLSPGK

SEQ ID NO: 79 - protein, 214 aa, Artificial sequence
  TIM-3 antibody light chain
EIVLTQSPATLSLSPGERATLSCRASQSVNDYLAWYQQKPGQAPRLLIYDASNRATGIPARFSGSGSGTDFTLTISSLEPEDFAVYYCQQGGHAPITFGQGTKVEIKRTVAAPSVFIFPPSDEQLKSGTASVVCLLNNFYPREAKVQWKVDNALQSGNSQESVTEQDSKDSTYSLSSTLTLSKADYEKHKVYACEVTHQGLSSPVTKSFNRGEC

SEQ ID NO: 80 - protein, 450 aa, Artificial sequence
  TIM-3 antibody heavy chain
EVQLVQSGAEVKKPGESLKISCKGSGYSFTSYWMQWVRQMPGKGLEWMGAIYPGDGDIRYTQNFKGQVTISADKSISTAYLQWSSLKASDTAMYYCARWEKSTTVVQRNYFDYWGQGTTVTVSSASTKGPSVFPLAPCSRSTSESTAALGCLVKDYFPEPVTVSWNSGALTSGVHTFPAVLQSSGLYSLSSVVTVPSSNFGTQTYTCNVDHKPSNTKVDKTVERKCCVECPPCPAPPAAASSVFLFPPKPKDTLMISRTPEVTCVVVDVSAEDPEVQFNWYVDGVEVHNAKTKPREEQFNSTFRVVSVLTVLHQDWLNGKEYKCKVSNKGLPSSIEKTISKTKGQPREPQVYTLPPSREEMTKNQVSLTCLVKGFYPSDIAVEWESNGQPENNYKTTPPMLDSDGSFFLYSRLTVDKSRWQQGNVFSCSVMHEALHNHYTQKSLSLSPGK

SEQ ID NO: 81 - protein, 213 aa, Artificial sequence
  TIM-3 antibody light chain
DIQMTQSPSSLSASVGDRVTITCKASENVGTFVSWYQQKPGKAPKLLIYGASNRYTGVPSRFSGSGSGTDFTLTISSLQPEDFATYYCGQSYSYPTFGQGTKLEIKRTVAAPSVFIFPPSDEQLKSGTASVVCLLNNFYPREAKVQWKVDNALQSGNSQESVTEQDSKDSTYSLSSTLTLSKADYEKHKVYACEVTHQGLSSPVTKSFNRGEC

SEQ ID NO: 82 - protein, 5 aa, Artificial sequence
  PD-1 HCDR1 genus
  1MISC_FEATURE (1)..(1): Xaa may be Ser or Asp
  1MISC_FEATURE (3)..(3): Xaa may be Val or Ala
  1MISC_FEATURE (5)..(5): Xaa may be His or Ser
XYXIX

SEQ ID NO: 83 - protein, 17 aa, Artificial sequence
  PD-1 HCDR2 genus
  MISC_FEATURE (6)..(6): Xaa may be Tyr or Phe
  MISC_FEATURE (7)..(7): Xaa may be Gly or Asp
GIIPIXXTANYAQKFQG

SEQ ID NO: 84 - protein, 14 aa, Artificial sequence
  PD-1 HCDR3 genus 1
  MISC_FEATURE (11)..(11): Xaa is Asn or Ser
PGLAAAYDTGXLDY

SEQ ID NO: 85 - protein, 11 aa, Artificial sequence
  PD-1 HCDR3 genus 2
  MISC_FEATURE (2)..(2): Xaa is Thr or Tyr
  MISC_FEATURE (3)..(3): Xaa is Leu or Val
  MISC_FEATURE (4)..(4): Xaa is Asp or Arg
  MISC_FEATURE (5)..(5): Xaa is Arg or Ala
  MISC_FEATURE (8)..(8): Xaa is His or Met
GXXXXTGXLDY

SEQ ID NO: 86 - protein, 11 aa, Artificial sequence
  PD-1 LCDR1 genus
  MISC_FEATURE (7)..(7): Xaa is Ser, Arg or Asp
  MISC_FEATURE (8)..(8): Xaa is Ser or Asn
RASQSVXXYLA

SEQ ID NO: 87 - protein, 7 aa, Artificial sequence
  PD-1 LCDR2 genus
  MISC_FEATURE (4)..(4): Xaa is Asn, Asp, Tyr, Ser or Thr
DASXRAT

SEQ ID NO: 88 - protein, 9 aa, Artificial sequence
  PD-1 LCDR3 genus
  MISC_FEATURE (4)..(4): Xaa is Ser, Asn, Gly, Glu, Asp, Trp or Ala
  MISC_FEATURE (5)..(5): Xaa is Asn, Tyr, Glu or Ala
QQRXXWPLT

SEQ ID NO: 89 - protein, 179 aa, Homo sapiens
SEVEYRAEVGQNAYLPCFYTPAAPGNLVPVCWGKGACPVFECGNVVLRTDERDVNYWTSRYWLNGDFRKGDVSLTIENVTLADSGIYCCRIQIPGIMNDEKFNLKLVIKPAKVTPAPTRQRDFTAAFPRMLTTRGHGPAETQTLGSLPDINLTQISTLANELRDSRLANDLRDSGATIR

SEQ ID NO: 90 - protein, 5 aa, Artificial sequence
  TIM-3 antibody HCDR1
NYWMS

SEQ ID NO: 91 - protein, 5 aa, Artificial sequence
  TIM-3 antibody HCDR1
SYAMS

SEQ ID NO: 92 - protein, 5 aa, Artificial sequence
  TIM-3 antibody HCDR1
GYWMH

SEQ ID NO: 93 - protein, 5 aa, Artificial sequence
  TIM-3 antibody HCDR1
DYWMS

SEQ ID NO: 94 - protein, 5 aa, Artificial sequence
  TIM-3 antibody HCDR1
SYVMY

SEQ ID NO: 95 - protein, 6 aa, Artificial sequence
  TIM-3 antibody HCDR1
SDYAWN

SEQ ID NO: 96 - protein, 5 aa, Artificial sequence
  TIM-3 antibody HCDR1
DTYLH

SEQ ID NO: 97 - protein, 5 aa, Artificial sequence
  TIM-3 antibody HCDR1
SYWMQ

SEQ ID NO: 98 - protein, 5 aa, Artificial sequence
  TIM-3 antibody HCDR1
SYGVH

SEQ ID NO: 99 - protein, 17 aa, Artificial sequence
  TIM-3 antibody HCDR2
AISGSGGSTYYADSVKG

SEQ ID NO: 100 - protein, 17 aa, Artificial sequence
  TIM-3 antibody HCDR2
AISYSGSSTYYADSVKG

SEQ ID NO: 101 - protein, 17 aa, Artificial sequence
  TIM-3 antibody HCDR2
VIKYSGGSKYYADSVKG

SEQ ID NO: 102 - protein, 17 aa, Artificial sequence
  TIM-3 antibody HCDR2
YINPYNDGTKYNEKFKG

SEQ ID NO: 103 - protein, 16 aa, Artificial sequence
  TIM-3 antibody HCDR2
YINYSGRTSYNPSLKS

SEQ ID NO: 104 - protein, 17 aa, Artificial sequence
  TIM-3 antibody HCDR2
RIDPTNGNIKYDPKFQG

SEQ ID NO: 105 - protein, 17 aa, Artificial sequence
  TIM-3 antibody HCDR2
AIYPGDGDIRYTQNFKG

SEQ ID NO: 106 - protein, 16 aa, Artificial sequence
  TIM-3 antibody HCDR2
VIWSDGSTTYNSALKS

SEQ ID NO: 107 - protein, 10 aa, Artificial sequence
  TIM-3 antibody HCDR2
DHWDPNFLDY

SEQ ID NO: 108 - protein, 8 aa, Artificial sequence
  TIM-3 antibody HCDR3
SPYAPLDY

SEQ ID NO: 109 - protein, 10 aa, Artificial sequence
  TIM-3 antibody HCDR3
NEEPDDRLDY

SEQ ID NO: 110 - protein, 7 aa, Artificial sequence
  TIM-3 antibody HCDR3
GTNWLDY

SEQ ID NO: 111 - protein, 8 aa, Artificial sequence
  TIM-3 antibody HCDR3
ELEGVFDY

SEQ ID NO: 112 - protein, 10 aa, Artificial sequence
  TIM-3 antibody HCDR3
DDYDVAPFAY

SEQ ID NO: 113 - protein, 6 aa, Artificial sequence
  TIM-3 antibody HCDR3
GGNFDY

SEQ ID NO: 114 - protein, 8 aa, Artificial sequence
  TIM-3 antibody HCDR3
PYYGFFDY

SEQ ID NO: 115 - protein, 15 aa, Artificial sequence
  TIM-3 antibody HCDR3
WEKSTTVVQRNYFDY

SEQ ID NO: 116 - protein, 12 aa, Artificial sequence
  TIM-3 antibody HCDR3
QANYRYDSAMDY

SEQ ID NO: 117 - protein, 12 aa, Artificial sequence
  TIM-3 antibody LCDR1
RASQSVSSSYLA

SEQ ID NO: 118 - protein, 11 aa, Artificial sequence
  TIM-3 antibody LCDR1
RASQSVNDYLA

SEQ ID NO: 119 - protein, 17 aa, Artificial sequence
  TIM-3 antibody LCDR1
KSSQSVLASSNNKNYLA

SEQ ID NO: 120 - protein, 12 aa, Artificial sequence
  TIM-3 antibody LCDR1
RASQSVSNSTLA

SEQ ID NO: 121 - protein, 15 aa, Artificial sequence
  TIM-3 antibody LCDR1
RASESLDSYGNSYIH

SEQ ID NO: 122 - protein, 11 aa, Artificial sequence
  TIM-3 antibody LCDR1
QATQDIVKNLN

SEQ ID NO: 123 - protein, 11 aa, Artificial sequence
  TIM-3 antibody LCDR1
KASQDVNTAVA

SEQ ID NO: 124 - protein, 11 aa, Artificial sequence
  TIM-3 antibody LCDR1
KASENVGTFVS

SEQ ID NO: 125 - protein, 15 aa, Artificial sequence
  TIM-3 antibody LCDR1
KASQSVDYDGDSYMN

SEQ ID NO: 126 - protein, 7 aa, Artificial sequence
  TIM-3 antibody LCDR2
GASSRAT

SEQ ID NO: 127 - protein, 7 aa, Artificial sequence
  TIM-3 antibody LCDR2
DASNRAT

SEQ ID NO: 128 - protein, 7 aa, Artificial sequence
  TIM-3 antibody LCDR2
WASTRES

SEQ ID NO: 129 - protein, 7 aa, Artificial sequence
  TIM-3 antibody LCDR2
TASSRAT

SEQ ID NO: 130 - protein, 7 aa, Artificial sequence
  TIM-3 antibody LCDR2
LASNLES

SEQ ID NO: 131 - protein, 7 aa, Artificial sequence
  TIM-3 antibody LCDR2
YVTELAE

SEQ ID NO: 132 - protein, 7 aa, Artificial sequence
  TIM-3 antibody LCDR2
SATYRYT

SEQ ID NO: 133 - protein, 7 aa, Artificial sequence
  TIM-3 antibody LCDR2
GASNRYT

SEQ ID NO: 134 - protein, 7 aa, Artificial sequence
  TIM-3 antibody LCDR2
TAANLQS

SEQ ID NO: 135 - protein, 9 aa, Artificial sequence
  TIM-3 antibody LCDR3
QQYGSSPLT

SEQ ID NO: 136 - protein, 9 aa, Artificial sequence
  TIM-3 antibody LCDR3
QQGGHAPIT

SEQ ID NO: 137 - protein, 9 aa, Artificial sequence
  TIM-3 antibody LCDR3
QQYYSTPLT

SEQ ID NO: 138 - protein, 280 aa, Homo sapiens
SEVEYRAEVGQNAYLPCFYTPAAPGNLVPVCWGKGACPVFECGNVVLRTDERDVNYWTSRYWLNGDFRKGDVSLTIENVTLADSGIYCCRIQIPGIMNDEKFNLKLVIKPAKVTPAPTRQRDFTAAFPRMLTTRGHGPAETQTLGSLPDINLTQISTLANELRDSRLANDLRDSGATIRIGIYIGAGICAGLALALIFGALIFKWYSHSKEKIQNLSLISLANLPPSGLANAVAEGIRSEENIYTIEENVYEVEEPNEYYCYVSSRQQPSQPLGCRFAMP

SEQ ID NO: 139 - protein, 9 aa, Artificial sequence
  TIM-3 antibody LCDR3
QQSYTSPWT

SEQ ID NO: 140 - protein, 9 aa, Artificial sequence
  TIM-3 antibody LCDR3
QQNNEDPFT

SEQ ID NO: 141 - protein, 9 aa, Artificial sequence
  TIM-3 antibody LCDR3
LQFYEFPLT

SEQ ID NO: 142 - protein, 9 aa, Artificial sequence
  TIM-3 antibody LCDR3
QQHYSTPYT

SEQ ID NO: 143 - protein, 8 aa, Artificial sequence
  TIM-3 antibody LCDR3
GQSYSYPT

SEQ ID NO: 144 - protein, 8 aa, Artificial sequence
  TIM-3 antibody LCDR3
GQSYSYPT

SEQ ID NO: 145 - protein, 119 aa, Artificial sequence
  TM3H21
EVQLLESGGGLVQPGGSLRLSCAASGFTFSNYWMSWVRQAPGKGLEWVSAISGSGGSTYYADSVKGRFTISRDNSKNTLYLQMNSLRAEDTAVYYCAKDHWDPNFLDYWGQGTLVTVSS

SEQ ID NO: 146 - protein, 117 aa, Artificial sequence
  TM3H24
EVQLLESGGGLVQPGGSLRLSCAASGFTFSSYAMSWVRQAPGKGLEWVSAISGSGGSTYYADSVKGRFTISRDNSKNTLYLQMNSLRAEDTAVYYCAKSPYAPLDYWGQGTLVTVSS

SEQ ID NO: 147 - protein, 116 aa, Artificial sequence
  TM3H30
EVQLLESGGGLVQPGGSLRLSCAASGFTFSGYWMHWVRQAPGKGLEWVSAISYSGSSTYYADSVKGRFTISRDNSKNTLYLQMNSLRAEDTAVYYCAKGTNWLDYWGQGTLVTVSS

SEQ ID NO: 148 - protein, 119 aa, Artificial sequence
  TM3H31
EVQLLESGGGLVQPGGSLRLSCAASGFTFSSYAMSWVRQAPGKGLEWVSAISGSGGSTYYADSVKGRFTISRDNSKNTLYLQMNSLRAEDTAVYYCAKNEEPDDRLDYWGQGTLVTVSS

SEQ ID NO: 149 - protein, 117 aa, Artificial sequence
  TM3H65
EVQLLESGGGLVQPGGSLRLSCAASGFTFSDYWMSWVRQAPGKGLEWVSVIKYSGGSKYYADSVKGRFTISRDNSKNTLYLQMNSLRAEDTAVYYCAKELEGVFDYWGQGTLVTVSS

SEQ ID NO: 150 - protein, 119 aa, Artificial sequence
  TM3H141
EVQLQQSGPELLKPGASVKMSCKASGYTFTSYVMYWVKQKPGQGLEWIGYINPYNDGTKYNEKFKGKATLTSDKSSSTAYMELSRLTSEDSAVYYCTRDDYDVAPFAYWGQGTLVTVSA

SEQ ID NO: 151 - protein, 115 aa, Artificial sequence
  TM3H96
DVQLQESGPGLVKPSQSLSLTCTVTGYSITSDYAWNWIRQFPGNKLEWMGYINYSGRTSYNPSLKSRISITRDTSKNQFFLQLNSVTTEDTATYYCTSGGNFDYWGQGTTLTVSS

SEQ ID NO: 152 - protein, 117 aa, Artificial sequence
  TM3H99
EVQLQQSGAELVKPGASVKLSCTASGFHIKDTYLHWVKQRPEQGLEWIGRIDPTNGNIKYDPKFQGKATITSDTSSNTAYLQLSSLTSEDTAVYYCARPYYGFFDYWGQGTTLTVSS

SEQ ID NO: 153 - protein, 130 aa, Artificial sequence
  TM3H144
EVQLQQSGAELARPGASVKLSCKASGYTFTSYWMQWVKQRPGQGLEWIGAIYPGDGDIRYTQNFKGKATLTADKSSSTAYMQLSSLASEDSAVYYCARWEKSTTVVQRNYFDYWGQGTTLTVSSCRRECT

SEQ ID NO: 154 - protein, 120 aa, Artificial sequence
  TM3H102
QVQLKESGPGLVAPSQSLSITCTISGFSLTSYGVHWVRQPPGKGLEWLVVIWSDGSTTYNSALKSRLSISKDNSKSQVFLKMNSLQTDDTAMYYCARQANYRYDSAMDYWGQGTSVTVSS

SEQ ID NO: 155 - protein, 108 aa, Artificial sequence
  PH9L1
EIVLTQSPGTLSLSPGERATLSCRASQSVSSSYLAWYQQKPGQAPRLLIYGASSRATGIPDRFSGSGSGTDFTLTISRLEPEDFAVYYCQQYGSSPLTFGQGTKVEIK

SEQ ID NO: 156 - protein, 107 aa, Artificial sequence
  TM3L33
EIVLTQSPATLSLSPGERATLSCRASQSVNDYLAWYQQKPGQAPRLLIYDASNRATGIPARFSGSGSGTDFTLTISSLEPEDFAVYYCQQGGHAPITFGQGTKVEIK

SEQ ID NO: 157 - protein, 113 aa, Artificial sequence
  PYYL6
DIVMTQSPDSLAVSLGERATINCKSSQSVLASSNNKNYLAWYQQKPGQPPKLLIYWASTRESGVPDRFSGSGSGTDFTLTISSLQAEDVAVYYCQQYYSTPLTFGQGTKVEIK

SEQ ID NO: 158 - protein, 108 aa, Artificial sequence
  TM3L12
EIVLTQSPGTLSLSPGERATLSCRASQSVSNSTLAWYQQKPGQAPRLLIYTASSRATGIPDRFSGSGSGTDFTLTISRLEPEDFAVYYCQQSYTSPWTFGQGTKVEIK

SEQ ID NO: 159 - protein, 111 aa, Artificial sequence
  TM3L61
DIVLTQSPASLAVSLGQRATISCRASESLDSYGNSYIHWYQQKPGQPPKLLIYLASNLESGVPARFSGSGSKTDFTLTIDPVEADDPATYYCQQNNEDPFTFGSGTKLEIK

SEQ ID NO: 160 - protein, 107 aa, Artificial sequence
  TM3L62
DIVMTQSPSSMSASLGDRITITCQATQDIVKNLNWYQQKPGKPPSFLIHYVTELAEGVPSRFSGSGSGSDYSLTISNLESEDFADYYCLQFYEFPLTFGAGTKLELK

SEQ ID NO: 161 - protein, 107 aa, Artificial sequence
  TM3L52
DIVMTQSHKFMSTSVGDRVSITCKASQDVNTAVAWYQQKPGQSPKLLIYSATYRYTGVPDRFTGSGSGTDFTFTISSVQAEDLAVYYCQQHYSTPYTFGSGTKLEIK

SEQ ID NO: 162 - protein, 105 aa, Artificial sequence
  TM3L67
DVQMIQSPKSMSMSVGERVTLSCKASENVGTFVSWYQQKPDQSPKLLIYGASNRYTGVPDRFTGSGSATDFTLTISSVQAEDLADYHCGQSYSYPTFGSGTKLEM

SEQ ID NO: 163 - protein, 111 aa, Artificial sequence
  TM3L64
DIQMTQSPASLAVSLGQRATISCKASQSVDYDGDSYMNWYQQKPGQPPKLLIYTAANLQSGIPARFSGSGSGTDFTLNIHPVEEEDAATYYCQQSNEDPFTFGSGTKLEIK

SEQ ID NO: 164 - protein, 5 aa, Artificial sequence
  TIM-3 HCDR1 genus
  MISC_FEATURE (1)..(1): Xaa is Asn, Ser, Gly or Asp
  MISC_FEATURE (3)..(3): Xaa is Trp or Ala
  MISC_FEATURE (5)..(5): Xaa is Ser or His
XYXMX

SEQ ID NO: 165 - protein, 17 aa, Artificial sequence
  TIM-3 HCDR2 genus
  MISC_FEATURE (1)..(1): Xaa is Ala or Val
  MISC_FEATURE (3)..(3): Xaa is Ser or Lys
  MISC_FEATURE (4)..(4): Xaa is Gly or Tyr
  MISC_FEATURE (9)..(9): Xaa is Thr or Lys
XIXXSGGSXYYADSVKG

SEQ ID NO: 166 - protein, 10 aa, Artificial sequence
  TIM-3 HCDR3 genus
  MISC_FEATURE (1)..(1): Xaa is Asp, Ser, Asn, Gly or Glu
  MISC_FEATURE (2)..(2): Xaa is His, Pro, Glu, Thr or Leu
  MISC_FEATURE (3)..(3): Xaa isTrp, Glu, Asn or deleted
  MISC_FEATURE (4)..(4): Xaa is Asp, Pro, or depeted
  MISC_FEATURE (5)..(5): Xaa is Pro, Tyr, Asp or deleted
  MISC_FEATURE (6)..(6): Xaa is Asn, Ala, Asp, Gly or deleted
  MISC_FEATURE (7)..(7): Xaa is Phe, Pro, Arg, Trp or Val
  MISC_FEATURE (8)..(8): Xaa is Leu or Phe
XXXXXXXXDY

SEQ ID NO: 167 - protein, 17 aa, Artificial sequence
  TIM-3 LCDR1 genus
  MISC_FEATURE (1)..(1): Xaa is Arg or Lys
  MISC_FEATURE (2)..(2): Xaa is Ala or Ser
  MISC_FEATURE (7)..(7): Xaa is Ser, Asn or Leu
  MISC_FEATURE (8)..(8): Xaa is Ser, Ala, Asn or deleted
  MISC_FEATURE (9)..(9): Xaa is Ser or deleted
  MISC_FEATURE (10)..(10): Xaa is Ser or deleted
  MISC_FEATURE (11)..(11): Xaa is Asn or deleted
  MISC_FEATURE (12)..(12): Xaa is Asn or deleted
  MISC_FEATURE (13)..(13): Xaa is Lys or deleted
  MISC_FEATURE (14)..(14): Xaa is Ser, Asn or Asp
  MISC_FEATURE (15)..(15): Xaa is Tyr or Thr
XXSQSVXXXXXXXXXLA

SEQ ID NO: 168 - protein, 7 aa, Artificial sequence
  TIM-3 LCDR2 genus
  MISC_FEATURE (1)..(1): Xaa is Gly, Asp, Trp or Thr
  MISC_FEATURE (4)..(4): Xaa is Ser, Asn or Thr
  MISC_FEATURE (6)..(6): Xaa is Ala or Glu
  MISC_FEATURE (7)..(7): Xaa is Thr or Ser
XASXRXX

SEQ ID NO: 169 - protein, 9 aa, Artificial sequence
  TIM-3 LCDR3 genus
  MISC_FEATURE (3)..(3): Xaa is Tyr, Gly or Ser
  MISC_FEATURE (4)..(4): Xaa is Gly or Tyr
  MISC_FEATURE (5)..(5): Xaa is Ser, His or Thr
  MISC_FEATURE (6)..(6): Xaa is Ser, Ala or Thr
  MISC_FEATURE (8)..(8): Xaa is Leu, Ile or Trp
QQXXXXPXT

SEQ ID NO: 170 - protein, 98 aa, Homo sapiens
QVQLVQSGAEVKKPGSSVKVSCKASGGTFSSYAISWVRQAPGQGLEWMGGIIPIFGTANYAQKFQGRVTITADESTSTAYMELSSLRSEDTAVYYCAR

SEQ ID NO: 171 - protein, 95 aa, Homo sapiens
EIVLTQSPATLSLSPGERATLSCRASQSVSSYLAWYQQKPGQAPRLLIYDASNRATGIPARFSGSGSGTDFTLTISSLEPEDFAVYYCQQRSNWP

SEQ ID NO: 172 - protein, 124 aa, Artificial sequence
  TM3H162
EVQLVQSGAEVKKPGESLKISCKGSGYSFTSYWMQWVRQMPGKGLEWMGAIYPGDGDIRYTQNFKGQVTISADKSISTAYLQWSSLKASDTAMYYCARWEKSTTVVQRNYFDYWGQGTTVTVSS

SEQ ID NO: 173 - protein, 106 aa, Artificial sequence
  TM3L85
DIQMTQSPSSLSASVGDRVTITCKASENVGTFVSWYQQKPGKAPKLLIYGASNRYTGVPSRFSGSGSGTDFTLTISSLQPEDFATYYCGQSYSYPTFGQGTKLEIK

SEQ ID NO: 174 - protein, 98 aa, Homo sapiens
EVQLLESGGGLVQPGGSLRLSCAASGFTFSSYAMSWVRQAPGKGLEWVSAISGSGGSTYYADSVKGRFTISRDNSKNTLYLQMNSLRAEDTAVYYCAK

SEQ ID NO: 175 - protein, 98 aa, Homo sapiens
QVQLVQSGAEVKKPGASVKVSCKASGYTFTGYYMHWVRQAPGQGLEWMGRINPNSGGTNYAQKFQGRVTSTRDTSISTAYMELSRLRSDDTVVYYCAR

SEQ ID NO: 176 - protein, 99 aa, Homo sapiens
QVQLQESGPGLVKPSQTLSLTCTVSGGSISSGDYYWSWIRQPPGKGLEWIGYIYYSGSTYYNPSLKSRVTISVDTSKNQFSLKLSSVTAADTAVYYCAR

SEQ ID NO: 177 - protein, 98 aa, Homo sapiens
QVQLVQSGAEVKKPGASVKVSCKASGYTFTSYAMHWVRQAPGQRLEWMGWINAGNGNTKYSQKFQGRVTITRDTSASTAYMELSSLRSEDTAVYYCAR

SEQ ID NO: 178 - protein, 100 aa, Homo sapiens
QVTLKESGPVLVKPTETLTLTCTVSGFSLSNARMGVSWIRQPPGKALEWLAHIFSNDEKSYSTSLKSRLTISKDTSKSQVVLTMTNMDPVDTATYYCARI

SEQ ID NO: 179 - protein, 98 aa, Homo sapiens
EVQLVQSGAEVKKPGESLKISCKGSGYSFTSYWIGWVRQMPGKGLEWMGIIYPGDSDTRYSPSFQGQVTISADKSISTAYLQWSSLKASDTAMYYCAR

SEQ ID NO: 180 - protein, 96 aa, Homo sapiens
EIVLTQSPGTLSLSPGERATLSCRASQSVSSSYLAWYQQKPGQAPRLLIYGASSRATGIPDRFSGSGSGTDFTLTISRLEPEDFAVYYCQQYGSSP

SEQ ID NO: 181 - protein, 96 aa, Homo sapiens; identical to SEQ ID NO: 180

SEQ ID NO: 182 - protein, 96 aa, Homo sapiens
DIQMTQSPSSLSASVGDRVTITCRASQSISSYLNWYQQKPGKAPKLLIYAASSLQSGVPSRFSGSGSGTDFTLTISSLQPEDFATYYCQQSYSTPI

SEQ ID NO: 183 - protein, 95 aa, Homo sapiens
DIQMTQSPSSLSASVGDRVTITCQASQDISNYLNWYQQKPGKAPKLLIYDASNLETGVPSRFSGSGSGTDFTFTISSLQPEDIATYYCQQYDNLP

SEQ ID NO: 184 - protein, 127 aa, Artificial sequence
  VH of gp120 binding mAb
QVQLVQSGAEVKKPGASVKVSCQASGYRFSNFVIHWVRQAPGQRFEWMGWINPYNGNKEFSAKFQDRVTFTADTSANTAYMELRSLRSADTAVYYCARVGPYSWDDSPQDNYYMDVWGKGTTVIVSS

SEQ ID NO: 185 - protein, 108 aa, Artificial sequence
  VL of gp120 binding mAb
EIVLTQSPGTLSLSPGERATFSCRSSHSIRSRRVAWYQHKPGQAPRLVIHGVSNRASGISDRFSGSGSGTDFTLTITRVEPEDFALYYCQVYGASSYTFGQGTKLERK

SEQ ID NO: 186 - protein, 449 aa, Artificial sequence
  Bispecific mAb HC1
QVQLVQSGAEVKKPGSSVKVSCKASGGTFSSYAISWVRQAPGQGLEWMGGIIPIFDTANYAQKFQGRVTITADESTSTAYMELSSLRSEDTAVYYCARPGLAAAYDTGSLDYWGQGTLVTVSSASTKGPSVFPLAPCSRSTSESTAALGCLVKDYFPEPVTVSWNSGALTSGVHTFPAVLQSSGLYSLSSVVTVTSSNFGTQTYTCNVDHKPSNTKVDKTVERKCCVECPPCPAPPAAASSVFLFPPKPKDTLMISRTPEVTCVVVDVSAEDPEVQFNWYVDGVEVHNAKTKPREEQFNSTFRVVSVLTVLHQDWLNGKEYKCKVSNKGLPSSIEKTISKTKGQPREPQVYTLPPSREEMTKNQVSLTCLVKGFYPSDIAVEWESNGQPENNYKTTPPMLDSDGSFLLYSKLTVDKSRWQQGNVFSCSVMHEALHNHYTQKSLSLSPGK

SEQ ID NO: 187 - protein, 443 aa, Artificial sequence
  Bispecific mAb HC1
EVQLVESGGGLVQPGGSLRLSCAASGFAFSRYDMSWVRQAPGKGLESVAYISGGGANTYYLDNVKGRFTISRDNAKNSLYLQMNSLRAEDTAVYYCASPYLSYFDVWGQGTLVTVSSASTKGPSVFPLAPCSRSTSESTAALGCLVKDYFPEPVTVSWNSGALTSGVHTFPAVLQSSGLYSLSSVVTVTSSNFGTQTYTCNVDHKPSNTKVDKTVERKCCVECPPCPAPPAAASSVFLFPPKPKDTLMISRTPEVTCVVVDVSAEDPEVQFNWYVDGVEVHNAKTKPREEQFNSTFRVVSVLTVLHQDWLNGKEYKCKVSNKGLPSSIEKTISKTKGQPREPQVYTLPPSREEMTKNQVSLTCLVKGFYPSDIAVEWESNGQPENNYKTTPPMLDSDGSFLLYSKLTVDKSRWQQGNVFSCSVMHEALHNHYTQKSLSLSPGK

SEQ ID NO: 188 - protein, 214 aa, Artificial sequence; identical to SEQ ID NO: 73
  Bispecific mAb LC1

SEQ ID NO: 189 - protein, 214 aa, Artificial sequence; identical to SEQ ID NO: 75
  Bispecific mAb LC1

SEQ ID NO: 190 - protein, 450 aa, Artificial sequence
  Bispecific mAb HC2
EVQLQQSGAELARPGASVKLSCKASGYTFTSYWMQWVKQRPGQGLEWIGAIYPGDGDIRYTQNFKGKATLTADKSSSTAYMQLSSLASEDSAVYYCARWEKSTTVVQRNYFDYWGQGTTLTVSSASTKGPSVFPLAPCSRSTSESTAALGCLVKDYFPEPVTVSWNSGALTSGVHTFPAVLQSSGLYSLSSVVTVTSSNFGTQTYTCNVDHKPSNTKVDKTVERKCCVECPPCPAPPAAASSVFLFPPKPKDTLMISRTPEVTCVVVDVSAEDPEVQFNWYVDGVEVHNAKTKPREEQFNSTFRVVSVLTVLHQDWLNGKEYKCKVSNKGLPSSIEKTISKTKGQPREPQVYTLPPSREEMTKNQVSLTCLVKGFYPSDIAVEWESNGQPENNYKTTPPMLDSDGSFFLYSRLTVDKSRWQQGNVFSCSVMHEALHNHYTQKSLSLSPGK

SEQ ID NO: 191 - protein, 443 aa, Artificial sequence
  Bispecific mAb HC2
EVQLLESGGGLVQPGGSLRLSCAASGFTFSSYAMSWVRQAPGKGLEWVSAISGSGGSTYYADSVKGRFTISRDNSKNTLYLQMNSLRAEDTAVYYCAKSPYAPLDYWGQGTLVTVSSASTKGPSVFPLAPCSRSTSESTAALGCLVKDYFPEPVTVSWNSGALTSGVHTFPAVLQSSGLYSLSSVVTVTSSNFGTQTYTCNVDHKPSNTKVDKTVERKCCVECPPCPAPPAAASSVFLFPPKPKDTLMISRTPEVTCVVVDVSAEDPEVQFNWYVDGVEVHNAKTKPREEQFNSTFRVVSVLTVLHQDWLNGKEYKCKVSNKGLPSSIEKTISKTKGQPREPQVYTLPPSREEMTKNQVSLTCLVKGFYPSDIAVEWESNGQPENNYKTTPPMLDSDGSFFLYSRLTVDKSRWQQGNVFSCSVMHEALHNHYTQKSLSLSPGK

SEQ ID NO: 192 - protein, 450 aa, Artificial sequence
  Bispecific mAb HC2
EVQLVQSGAEVKKPGESLKISCKGSGYSFTSYWMQWVRQMPGKGLEWMGAIYPGDGDIRYTQNFKGQVTISADKSISTAYLQWSSLKASDTAMYYCARWEKSTTVVQRNYFDYWGQGTTVTVSSASTKGPSVFPLAPCSRSTSESTAALGCLVKDYFPEPVTVSWNSGALTSGVHTFPAVLQSSGLYSLSSVVTVTSSNFGTQTYTCNVDHKPSNTKVDKTVERKCCVECPPCPAPPAAASSVFLFPPKPKDTLMISRTPEVTCVVVDVSAEDPEVQFNWYVDGVEVHNAKTKPREEQFNSTFRVVSVLTVLHQDWLNGKEYKCKVSNKGLPSSIEKTISKTKGQPREPQVYTLPPSREEMTKNQVSLTCLVKGFYPSDIAVEWESNGQPENNYKTTPPMLDSDGSFFLYSRLTVDKSRWQQGNVFSCSVMHEALHNHYTQKSLSLSPGK

SEQ ID NO: 193 - protein, 213 aa, Artificial sequence
  Bispecific mAb LC2
DVQMIQSPKSMSMSVGERVTLSCKASENVGTFVSWYQQKPDQSPKLLIYGASNRYTGVPDRFTGSGSATDFTLTISSVQAEDLADYHCGQSYSYPTFGSGTKLEMKRTVAAPSVFIFPPSDEQLKSGTASVVCLLNNFYPREAKVQWKVDNALQSGNSQESVTEQDSKDSTYSLSSTLTLSKADYEKHKVYACEVTHQGLSSPVTKSFNRGEC

SEQ ID NO: 194 - protein, 214 aa, Artificial sequence; identical to SEQ ID NO: 79
  Bispecific mAb LC2

SEQ ID NO: 195 - protein, 213 aa, Artificial sequence; identical to SEQ ID NO: 81
  Bispecific mAb LC2

SEQ ID NO: 196 - DNA, 369 bp, Artificial sequence
  DNA of PD1H170
caggtgcagctggtgcagagcggcgcggaagtgaaaaaaccgggcagcagcgtgaaagtgagctgcaaagcgagcggcggcacctttagcagctatgcgattagctgggtgcgccaggcgccgggccagggcctggaatggatgggcggcattattccgatttttgacaccgcgaactatgcgcagaaatttcagggccgcgtgaccattaccgcggatgaaagcaccagcaccgcgtatatggaactgagcagcctgcgcagcgaagataccgcggtgtattattgcgcgcgccctggtctcgctgcggcttatgatactggttccttggactattggggccagggcaccctggtgaccgtgagcagc

SEQ ID NO: 197 - DNA, 321 bp, Artificial sequence
  DNA of PD1L148
gaaattgtgctgacccagagcccggcgaccctgagcctgagcccgggcgaacgcgcgaccctgagctgccgcgcgagccagagcgttcgctcctacctggcgtggtatcagcagaaaccgggccaggcgccgcgcctgctgatctacgacgcgagcaatcgtgcgaccggcattccggcgcgctttagcggctccggtagcggcaccgattttaccctgaccattagcagcctggaaccggaagattttgcggtgtattattgccagcaacgtaattattggccgctgacctttggccagggcaccaaagtggaaattaaa

SEQ ID NO: 198 - DNA, 351 bp, Artificial sequence
  DNA of PD1H129
gaagtgcagctggtggaatctggcggcggactggtgcagcctggcggatctctgagactgagctgtgccgccagcggcttcgccttcagcagatacgacatgagctgggtgcgccaggcccctggcaaaggactggaaagcgtggcctacatctctggcggaggcgccaacacctactacctggacaacgtgaagggccggttcaccatcagccgggacaacgccaagaacagcctgtacctgcagatgaactccctgcgggccgaggacaccgccgtgtactattgcgcctccccctacctgagctacttcgacgtgtggggccagggcacactcgtgaccgtgtcatct

SEQ ID NO: 199 - DNA, 321 bp, Artificial sequence
  DNA of PD1L62
gagatcgtgatgacccagagccctgccaccctgtccgtgtctccaggcgaaagagccaccctgagctgcagagccagccagagcctgagcgactacctgcactggtatcagcagaagcccggccaggcccccagactgctgatcaagtctgccagccagtccatcagcggcatccccgccagattttctggcagcggctccggcaccgagttcaccctgacaatcagcagcctgcagagcgaggacttcgccgtgtactactgccagaacggccacagcttcccttacaccttcggccagggcaccaagctggaaatcaag

SEQ ID NO: 200 - DNA, 360 bp, Artificial sequence
  DNA of PD1H163
caggtgcagctggtgcagagcggcgcggaagtgaaaaaaccgggcagcagcgtgaaagtgagctgcaaagcgagcggcggcaccttcaagtcctatgtgattcattgggtgcgccaggcgccgggccagggcctggaatggatgggcggtattatcccaatttttggcaccgccaattatgcgcagaaatttcagggccgcgtgaccattaccgctgatgaaagcaccagcaccgcgtatatggaactgagcagcctgcgcagcgaagataccgcggtgtattattgcgcgcgcggttatgtgcgggctacgggcatgttggactattggggccagggcaccctggtgaccgtgagcagc

SEQ ID NO: 201 - DNA, 321 bp, Artificial sequence
  DNA of PD1L185
gaaattgtgctgacccagagcccggcgaccctgagcctgagcccgggcgaacgcgcgaccctgagctgccgcgcgagccagagcgttagcaattatctggcgtggtatcagcagaaaccgggccaggcgccgcgcctgctgatctacgacgccagcaatcgcgcgaccggcattccggcgcgctttagcggctccggtagcggcaccgattttaccctgaccattagcagcctggaaccggaagattttgcggtgtattattgccagcaacgtgcatattggccgctgacctttggccagggcaccaaagtggaaattaaa

SEQ ID NO: 202 - DNA, 360 bp, Artificial sequence
  DNA of PD1H164
caggtgcagctggtgcagagcggcgcggaagtgaaaaaaccgggcagcagcgtgaaagtgagctgcaaagcgagcggcggcaccttcagcgattatgtgatttcctgggtgcgccaggcgccgggccagggcctggaatggatgggcggtattatcccgatttacgggaccgctaactatgcgcagaaatttcagggccgcgtgaccattaccgctgatgaaagcaccagcaccgcgtatatggaactgagcagcctgcgcagcgaagataccgcggtgtattattgcgcgcgcggtaccctcgaccggaccgggcatttggactattggggccagggcaccctggtgaccgtgagcagc

SEQ ID NO: 203 - DNA, 321 bp, Artificial sequence
  DNA of PD1L86
gaaattgtgctgacccagagcccggcgaccctgagcctgagcccgggcgaacgcgcgaccctgagctgccgcgcgagccagagcgtctcctcctaccttgcgtggtatcagcagaaaccgggccaggcgccgcgcctgctgatccacgacgcctctacgcgtgcgaccggcattccggcgcgctttagcggctccggtagcggcaccgattttaccctgaccattagcagcctggaaccggaagattttgcggtgtattattgccagcaacgtaattattggccgctcacctttggccagggcaccaaagtggaaattaaa

SEQ ID NO: 204 - DNA, 351 bp, Artificial sequence
  DNA of TM3H24
gaagtgcagctgctggaaagcggcggcggcctggtgcagccgggcggcagcctgcgcctgagctgcgcggcaagcggctttacctttagcagctatgcgatgagctgggtgcgccaggcgccgggcaaaggcctggaatgggtgagcgcgattagcggcagcggcggcagcacctattatgcggatagcgtgaaaggccgctttaccattagccgcgataacagcaaaaacaccctgtatctgcagatgaacagcctgcgcgcggaagataccgcggtgtattattgcgcgaaatccccgtacgcgcccttggactattggggccagggcaccctggtgaccgtgagcagc

SEQ ID NO: 205 - DNA, 321 bp, Artificial sequence
  DNA of TM3L33
gaaattgtgctgacccagagcccggcgaccctgagcctgagcccgggcgaacgcgcgacccttagctgccgtgcaagtcagagtgtgaacgactacctggcgtggtatcagcagaaaccgggccaggcgccgcgcctgctgatttatgatgcgagcaaccgcgcgaccggcattccggcgcgctttagcggcagcggcagcggcaccgattttaccctgaccattagcagcctggaaccggaagattttgcggtgtattattgccagcagggtggtcacgcgccgatcacctttggccagggcaccaaagtggaaattaaa

SEQ ID NO: 206 - DNA, 372 bp, Artificial sequence
  DNA of TM3H162
gaagtgcagctggtgcagtctggcgccgaagtgaagaagcctggcgagagcctgaagatcagctgcaagggcagcggctacagcttcaccagctactggatgcagtgggtgcgccagatgcctggcaagggcctggaatggatgggcgccatctatcccggcgacggcgacatcagatacacccagaacttcaagggccaagtgaccatcagcgccgacaagagcatcagcaccgcctacctgcagtggtccagcctgaaggccagcgacaccgccatgtactactgtgccagatgggagaagtccaccaccgtggtgcagcggaactacttcgactactggggccagggcaccacagtgaccgtgtctagt

SEQ ID NO: 207 - DNA, 318 bp, Artificial sequence
  DNA of TM3L85
gacatccagatgacccagagccccagcagcctgtctgccagcgtgggcgacagagtgaccatcacatgcaaggccagcgagaacgtgggcaccttcgtgtcctggtatcagcagaagcccggcaaggcccccaagctgctgatctacggcgccagcaacagatacaccggcgtgcccagcagattcagcggctctggcagcggcaccgacttcaccctgaccatctctagcctgcagcccgaggacttcgccacctactactgcggccagagctacagctaccccacctttggccagggcaccaagctggaaatcaag

SEQ ID NO: 208 - DNA, 357 bp, Artificial sequence
  DNA of TM3H21
gaagtgcagctgctggaaagcggcggcggcctggtgcagccgggcggcagcctgcgcctgagctgcgcggcgagcggctttacctttagcaactattggatgagctgggtgcgccaggcgccgggcaaaggcctggaatgggtgagcgcgattagcggcagcggcggcagcacctattatgcggatagcgtgaaaggccgctttaccattagccgcgataacagcaaaaacaccctgtatctgcagatgaacagcctgcgcgcggaagataccgcggtgtattattgcgcgaaagatcattgggatcccaattttttggactattggggccagggcaccctggtgaccgtgagcagc

SEQ ID NO: 209 - DNA, 324 bp, Artificial sequence
  DNA of PH9L1
gaaattgtgctgacccagagcccgggcaccctgagcctgagcccgggcgaacgcgcgaccctgagctgccgcgcgagccagagcgtgagcagcagctatctggcgtggtatcagcagaaaccgggccaggcgccgcgcctgctgatttatggcgcgagcagccgcgcgaccggcattccggatcgctttagcggcagcggcagcggcaccgattttaccctgaccattagccgcctggaaccggaagattttgcggtgtattattgccagcagtatggcagcagcccgctgacctttggccagggcaccaaagtggaaattaaa

SEQ ID NO: 210 - DNA, 351 bp, Artificial sequence
  DNA of TM3H65
gaagtgcagctgctggaaagcggcggcggcctggtgcagccgggcggcagcctgcgcctgagctgcgcggcgagcggctttacctttagcgactattggatgagctgggtgcgccaggcgccgggcaaaggcctggaatgggtgagcgtgatcaagtatagcggtggctccaaatattatgcggatagcgtgaaaggccgctttaccattagccgcgataacagcaaaaacaccctgtatctgcagatgaacagcctgcgcgcggaagataccgcggtgtattattgcgcgaaagagctggagggggtgttcgactattggggccagggcaccctggtgaccgtgagcagc

SEQ ID NO: 211 - DNA, 324 bp, Artificial sequence
  DNA of TM3L12
gaaattgtgctgacccagagcccgggcaccctgagcctgagcccgggcgaacgcgcgaccctgagctgccgcgcgagccagagcgttagcaatagcactctggcgtggtatcagcagaaaccgggccaggcgccgcgcctgctgatttatactgcgagcagccgcgcgaccggcattccggatcgctttagcggcagcggcagcggcaccgattttaccctgaccattagccgcctggaaccggaagattttgcggtgtattattgccagcagtcttacacatctccgtggacttttggccagggcaccaaagtggaaattaaa

SEQ ID NO: 212 - protein, 449 aa, Artificial sequence
  HC of PD1B114
QVQLVQSGAEVKKPGSSVKVSCKASGGTFSSYAISWVRQAPGQGLEWMGGIIPIFGTANYAQKFQGRVTITADESTSTAYMELSSLRSEDTAVYYCARPGLAAAYDTGNLDYWGQGTLVTVSSASTKGPSVFPLAPCSRSTSESTAALGCLVKDYFPEPVTVSWNSGALTSGVHTFPAVLQSSGLYSLSSVVTVTSSNFGTQTYTCNVDHKPSNTKVDKTVERKCCVECPPCPAPPAAASSVFLFPPKPKDTLMISRTPEVTCVVVDVSAEDPEVQFNWYVDGVEVHNAKTKPREEQFNSTFRVVSVLTVLHQDWLNGKEYKCKVSNKGLPSSIEKTISKTKGQPREPQVYTLPPSREEMTKNQVSLTCLVKGFYPSDIAVEWESNGQPENNYKTTPPMLDSDGSFFLYSKLTVDKSRWQQGNVFSCSVMHEALHNHYTQKSLSLSPGK

SEQ ID NO: 213 - protein, 214 aa, Artificial sequence
  LC of PD1B114
EIVLTQSPATLSLSPGERATLSCRASQSVSSYLAWYQQKPGQAPRLLIYDASNRATGIPARFSGSGSGTDFTLTISSLEPEDFAVYYCQQRSNWPLTFGQGTKVEIKRTVAAPSVFIFPPSDEQLKSGTASVVCLLNNFYPREAKVQWKVDNALQSGNSQESVTEQDSKDSTYSLSSTLTLSKADYEKHKVYACEVTHQGLSSPVTKSFNRGEC

SEQ ID NO: 214 - protein, 449 aa, Artificial sequence; identical to SEQ ID NO: 212
  HC of PD1B149

SEQ ID NO: 215 - protein, 214 aa, Artificial sequence
  LC of PD1B149
EIVLTQSPATLSLSPGERATLSCRASQSVRNYLAWYQQKPGQAPRLLIHDASNRATGIPARFSGSGSGTDFTLTISSLEPEDFAVYYCQQRNYWPLTFGQGTKVEIKRTVAAPSVFIFPPSDEQLKSGTASVVCLLNNFYPREAKVQWKVDNALQSGNSQESVTEQDSKDSTYSLSSTLTLSKADYEKHKVYACEVTHQGLSSPVTKSFNRGEC

SEQ ID NO: 216 - protein, 449 aa, Artificial sequence
  HC of PD1B160
QVQLVQSGAEVKKPGSSVKVSCKASGGTFSSYAISWVRQAPGQGLEWMGGIIPIFDTANYAQKFQGRVTITADESTSTAYMELSSLRSEDTAVYYCARPGLAAAYDTGNLDYWGQGTLVTVSSASTKGPSVFPLAPCSRSTSESTAALGCLVKDYFPEPVTVSWNSGALTSGVHTFPAVLQSSGLYSLSSVVTVTSSNFGTQTYTCNVDHKPSNTKVDKTVERKCCVECPPCPAPPAAASSVFLFPPKPKDTLMISRTPEVTCVVVDVSAEDPEVQFNWYVDGVEVHNAKTKPREEQFNSTFRVVSVLTVLHQDWLNGKEYKCKVSNKGLPSSIEKTISKTKGQPREPQVYTLPPSREEMTKNQVSLTCLVKGFYPSDIAVEWESNGQPENNYKTTPPMLDSDGSFFLYSKLTVDKSRWQQGNVFSCSVMHEALHNHYTQKSLSLSPGK

SEQ ID NO: 217 - protein, 214 aa, Artificial sequence
  LC of PD1B160
EIVLTQSPATLSLSPGERATLSCRASQSVDSYLAWYQQKPGQAPRLLIKDASDRATGIPARFSGSGSGTDFTLTISSLEPEDFAVYYCQQRGNWPLTFGQGTKVEIKRTVAAPSVFIFPPSDEQLKSGTASVVCLLNNFYPREAKVQWKVDNALQSGNSQESVTEQDSKDSTYSLSSTLTLSKADYEKHKVYACEVTHQGLSSPVTKSFNRGEC

SEQ ID NO: 218 - protein, 449 aa, Artificial sequence; identical to SEQ ID NO: 216
  HC of PD1B162

SEQ ID NO: 219 - protein, 214 aa, Artificial sequence
  LC of PD1B162
EIVLTQSPATLSLSPGERATLSCRASQSVDSYLAWYQQKPGQAPRLLIYDASNRATGIPARFSGSGSGTDFTLTISSLEPEDFAVYYCQQREYWPLTFGQGTKVEIKRTVAAPSVFIFPPSDEQLKSGTASVVCLLNNFYPREAKVQWKVDNALQSGNSQESVTEQDSKDSTYSLSSTLTLSKADYEKHKVYACEVTHQGLSSPVTKSFNRGEC

SEQ ID NO: 220 - protein, 449 aa, Artificial sequence; identical to SEQ ID NO: 216
  HC of PD1B164

SEQ ID NO: 221 - protein, 214 aa, Artificial sequence
  LC of PD1B164
EIVLTQSPATLSLSPGERATLSCRASQSVRSYLAWYQQKPGQAPRLLIYDASYRATGIPARFSGSGSGTDFTLTISSLEPEDFAVYYCQQRDYWPLTFGQGTKVEIKRTVAAPSVFIFPPSDEQLKSGTASVVCLLNNFYPREAKVQWKVDNALQSGNSQESVTEQDSKDSTYSLSSTLTLSKADYEKHKVYACEVTHQGLSSPVTKSFNRGEC

SEQ ID NO: 222 - protein, 449 aa, Artificial sequence
  HC of PD1B183
QVQLVQSGAEVKKPGSSVKVSCKASGGTFSSYAISWVRQAPGQGLEWMGGIIPIFGTANYAQKFQGRVTITADESTSTAYMELSSLRSEDTAVYYCARPGLAAAYDTGSLDYWGQGTLVTVSSASTKGPSVFPLAPCSRSTSESTAALGCLVKDYFPEPVTVSWNSGALTSGVHTFPAVLQSSGLYSLSSVVTVTSSNFGTQTYTCNVDHKPSNTKVDKTVERKCCVECPPCPAPPAAASSVFLFPPKPKDTLMISRTPEVTCVVVDVSAEDPEVQFNWYVDGVEVHNAKTKPREEQFNSTFRVVSVLTVLHQDWLNGKEYKCKVSNKGLPSSIEKTISKTKGQPREPQVYTLPPSREEMTKNQVSLTCLVKGFYPSDIAVEWESNGQPENNYKTTPPMLDSDGSFFLYSKLTVDKSRWQQGNVFSCSVMHEALHNHYTQKSLSLSPGK

SEQ ID NO: 223 - protein, 214 aa, Artificial sequence
  LC of PD1B183
EIVLTQSPATLSLSPGERATLSCRASQSVSSYLAWYQQKPGQAPRLLIKDASNRATGIPARFSGSGSGTDFTLTISSLEPEDFAVYYCQQRGYWPLTFGQGTKVEIKRTVAAPSVFIFPPSDEQLKSGTASVVCLLNNFYPREAKVQWKVDNALQSGNSQESVTEQDSKDSTYSLSSTLTLSKADYEKHKVYACEVTHQGLSSPVTKSFNRGEC

SEQ ID NO: 224 - protein, 449 aa, Artificial sequence; identical to SEQ ID NO: 222
  HC of PD1B184

SEQ ID NO: 225 - protein, 214 aa, Artificial sequence; identical to SEQ ID NO: 215
  LC of PD1B184

SEQ ID NO: 226 - protein, 449 aa, Artificial sequence; identical to SEQ ID NO: 222
  HC of PD1B185

SEQ ID NO: 227 - protein, 214 aa, Artificial sequence
  LC of PD1B185
EIVLTQSPATLSLSPGERATLSCRASQSVRNYLAWYQQKPGQAPRLLIYDASDRATGIPARFSGSGSGTDFTLTISSLEPEDFAVYYCQQRWNWPLTFGQGTKVEIKRTVAAPSVFIFPPSDEQLKSGTASVVCLLNNFYPREAKVQWKVDNALQSGNSQESVTEQDSKDSTYSLSSTLTLSKADYEKHKVYACEVTHQGLSSPVTKSFNRGEC

SEQ ID NO: 228 - protein, 449 aa, Artificial sequence; identical to SEQ ID NO: 222
  HC of PD1B192

SEQ ID NO: 229 - protein, 214 aa, Artificial sequence
  LC or PD1B192
EIVLTQSPATLSLSPGERATLSCRASQSVDSYLAWYQQKPGQAPRLLIHDASNRATGIPARFSGSGSGTDFTLTISSLEPEDFAVYYCQQRNYWPLTFGQGTKVEIKRTVAAPSVFIFPPSDEQLKSGTASVVCLLNNFYPREAKVQWKVDNALQSGNSQESVTEQDSKDSTYSLSSTLTLSKADYEKHKVYACEVTHQGLSSPVTKSFNRGEC

SEQ ID NO: 230 - protein, 120 aa, Artificial sequence [sequence omitted]

SEQ ID NO: 231 - protein, 111 aa, Artificial sequence [sequence omitted]

SEQ ID NO: 232 - protein, 113 aa, Artificial sequence [sequence omitted]

SEQ ID NO: 233 - protein, 107 aa, Artificial sequence [sequence omitted]

SEQ ID NO: 234 - protein, 121 aa, Artificial sequence
  Durvalumab VH
EVQLVESGGGLVQPGGSLRLSCAASGFTFSRYWMSWVRQAPGKGLEWVANIKQDGSEKYYVDSVKGRFTISRDNAKNSLYLQMNSLRAEDTAVYYCAREGGWFGELAFDYWGQGTLVTVSS

SEQ ID NO: 235 - protein, 108 aa, Artificial sequence
  Durvalumab VL
EIVLTQSPGTLSLSPGERATLSCRASQRVSSSYLAWYQQKPGQAPRLLIYDASSRATGIPDRFSGSGSGTDFTLTISRLEPEDFAVYYCQQYGSLPWTFGQGTKVEIK

SEQ ID NO: 236 - protein, 118 aa, Artificial sequence [sequence omitted]

SEQ ID NO: 237 - protein, 107 aa, Artificial sequence [sequence omitted]

SEQ ID NO: 238 - protein, 120 aa, Artificial sequence
  Avelumab VH
EVQLLESGGGLVQPGGSLRLSCAASGFTFSSYIMMWVRQAPGKGLEWVSSIYPSGGITFYADTVKGRFTISRDNSKNTLYLQMNSLRAEDTAVYYCARIKLGTVTTVDYWGQGTLVTVSS

SEQ ID NO: 239 - protein, 110 aa, Artificial sequence
  Avelumab VL
QSALTQPASVSGSPGQSITISCTGTSSDVGGYNYVSWYQQHPGKAPKLMIYDVSNRPSGVSNRFSGSKSGNTASLTISGLQAEDEADYYCSSYTSSSTRVFGTGTKVTVL

SEQ ID NO: 240 - protein, 443 aa, Artificial Sequence
  TM3B105 Heavy chain
EVQLLESGGGLVQPGGSLRLSCAASGFTFSSYAMSWVRQAPGKGLEWVSAISGSGGSTYYADSVKGRFTISRDNSKNTLYLQMNSLRAEDTAVYYCAKSPYAPLDYWGQGTLVTVSSASTKGPSVFPLAPCSRSTSESTAALGCLVKDYFPEPVTVSWNSGALTSGVHTFPAVLQSSGLYSLSSVVTVTSSNFGTQTYTCNVDHKPSNTKVDKTVERKCCVECPPCPAPPAAASSVFLFPPKPKDTLMISRTPEVTCVVVDVSAEDPEVQFNWYVDGVEVHNAKTKPREEQFNSTFRVVSVLTVLHQDWLNGKEYKCKVSNKGLPSSIEKTISKTKGQPREPQVYTLPPSREEMTKNQVSLTCLVKGFYPSDIAVEWESNGQPENNYKTTPPMLDSDGSFFLYSKLTVDKSRWQQGNVFSCSVMHEALHNHYTQKSLSLSPGK

SEQ ID NO: 241 - protein, 449 aa, Artificial sequence
  Bispecific mAb HC1
QVQLVQSGAEVKKPGSSVKVSCKASGGTFSSYAISWVRQAPGQGLEWMGGIIPIFDTANYAQKFQGRVTITADESTSTAYMELSSLRSEDTAVYYCARPGLAAAYDTGSLDYWGQGTLVTVSSASTKGPSVFPLAPCSRSTSESTAALGCLVKDYFPEPVTVSWNSGALTSGVHTFPAVLQSSGLYSLSSVVTVPSSNFGTQTYTCNVDHKPSNTKVDKTVERKCCVECPPCPAPPVAGPSVFLFPPKPKDTLMISRTPEVTCVVVDVSHEDPEVQFNWYVDGVEVHNAKTKPREEQFNSTFRVVSVLTVVHQDWLNGKEYKCKVSNKGLPAPIEKTISKTKGQPREPQVYTLPPSREEMTKNQVSLTCLVKGFYPSDIAVEWESNGQPENNYKTTPPMLDSDGSFLLYSKLTVDKSRWQQGNVFSCSVMHEALHNHYTQKSLSLSPGK

SEQ ID NO: 242 - protein, 444 aa, Artificial sequence; identical to SEQ ID NO: 74
  Bispecific mAb HC1

SEQ ID NO: 243 - protein, 450 aa, Artificial sequence; identical to SEQ ID NO: 72
  Bispecific mAb HC1

SEQ ID NO: 244 - protein, 450 aa, Artificial sequence
  Bispecific mAb HC2
EVQLVQSGAEVKKPGESLKISCKGSGYSFTSYWMQWVRQMPGKGLEWMGAIYPGDGDIRYTQNFKGQVTISADKSISTAYLQWSSLKASDTAMYYCARWEKSTTVVQRNYFDYWGQGTTVTVSSASTKGPSVFPLAPCSRSTSESTAALGCLVKDYFPEPVTVSWNSGALTSGVHTFPAVLQSSGLYSLSSVVTVPSSNFGTQTYTCNVDHKPSNTKVDKTVERKCCVECPPCPAPPVAGPSVFLFPPKPKDTLMISRTPEVTCVVVDVSHEDPEVQFNWYVDGVEVHNAKTKPREEQFNSTFRVVSVLTVVHQDWLNGKEYKCKVSNKGLPAPIEKTISKTKGQPREPQVYTLPPSREEMTKNQVSLTCLVKGFYPSDIAVEWESNGQPENNYKTTPPMLDSDGSFFLYSRLTVDKSRWQQGNVFSCSVMHEALHNHYTQKSLSLSPGK

SEQ ID NO: 245 - protein, 443 aa, Artificial sequence
  Bispecific mAb HC2
EVQLLESGGGLVQPGGSLRLSCAASGFTFSSYAMSWVRQAPGKGLEWVSAISGSGGSTYYADSVKGRFTISRDNSKNTLYLQMNSLRAEDTAVYYCAKSPYAPLDYWGQGTLVTVSSASTKGPSVFPLAPCSRSTSESTAALGCLVKDYFPEPVTVSWNSGALTSGVHTFPAVLQSSGLYSLSSVVTVPSSNFGTQTYTCNVDHKPSNTKVDKTVERKCCVECPPCPAPPVAGPSVFLFPPKPKDTLMISRTPEVTCVVVDVSHEDPEVQFNWYVDGVEVHNAKTKPREEQFNSTFRVVSVLTVVHQDWLNGKEYKCKVSNKGLPAPIEKTISKTKGQPREPQVYTLPPSREEMTKNQVSLTCLVKGFYPSDIAVEWESNGQPENNYKTTPPMLDSDGSFFLYSRLTVDKSRWQQGNVFSCSVMHEALHNHYTQKSLSLSPGK

SEQ ID NO: 246 - protein, 444 aa, Artificial sequence
  Bispecific mAb HC2
EVQLLESGGGLVQPGGSLRLSCAASGFTFSSYAMSWVRQAPGKGLEWVSAISGSGGSTYYADSVKGRFTISRDNSKNTLYLQMNSLRAEDTAVYYCAKSPYAPLDYWGQGTLVTVSSASTKGPSVFPLAPCSRSTSESTAALGCLVKDYFPEPVTVSWNSGALTSGVHTFPAVLQSSGLYSLSSVVTVPSSSLGTKTYTCNVDHKPSNTKVDKRVESKYGPPCPPCPAPEFLGGPSVFLFPPKPKDTLMISRTPEVTCVVVDVSQEDPEVQFNWYVDGVEVHNAKTKPREEQFNSTYRVVSVLTVLHQDWLNGKEYKCKVSNKGLPSSIEKTISKAKGQPREPQVYTLPPSQEEMTKNQVSLTCLVKGFYPSDIAVEWESNGQPENNYKTTPPVLDSDGSFLLYSKLTVDKSRWQEGNVFSCSVMHEALHNHYTQKSLSLSLGK

SEQ ID NO: 247 - protein, 451 aa, Artificial sequence
  Bispecific mAb HC2
EVQLVQSGAEVKKPGESLKISCKGSGYSFTSYWMQWVRQMPGKGLEWMGAIYPGDGDIRYTQNFKGQVTISADKSISTAYLQWSSLKASDTAMYYCARWEKSTTVVQRNYFDYWGQGTTVTVSSASTKGPSVFPLAPCSRSTSESTAALGCLVKDYFPEPVTVSWNSGALTSGVHTFPAVLQSSGLYSLSSVVTVPSSSLGTKTYTCNVDHKPSNTKVDKRVESKYGPPCPPCPAPEFLGGPSVFLFPPKPKDTLMISRTPEVTCVVVDVSQEDPEVQFNWYVDGVEVHNAKTKPREEQFNSTYRVVSVLTVLHQDWLNGKEYKCKVSNKGLPSSIEKTISKAKGQPREPQVYTLPPSQEEMTKNQVSLTCLVKGFYPSDIAVEWESNGQPENNYKTTPPVLDSDGSFLLYSKLTVDKSRWQEGNVFSCSVMHEALHNHYTQKSLSLSLGK

SEQ ID NO: 248 - protein, 443 aa, Artificial sequence
  Bispecific mAb HC2
EVQLLESGGGLVQPGGSLRLSCAASGFTFSSYAMSWVRQAPGKGLEWVSAISGSGGSTYYADSVKGRFTISRDNSKNTLYLQMNSLRAEDTAVYYCAKSPYAPLDYWGQGTLVTVSSASTKGPSVFPLAPCSRSTSESTAALGCLVKDYFPEPVTVSWNSGALTSGVHTFPAVLQSSGLYSLSSVVTVPSSNFGTQTYTCNVDHKPSNTKVDKTVERKCCVECPPCPAPPAAASSVFLFPPKPKDTLMISRTPEVTCVVVDVSAEDPEVQFNWYVDGVEVHNAKTKPREEQFNSTFRVVSVLTVLHQDWLNGKEYKCKVSNKGLPSSIEKTISKTKGQPREPQVYTLPPSREEMTKNQVSLTCLVKGFYPSDIAVEWESNGQPENNYKTTPPMLDSDGSFFLYSRLTVDKSRWQQGNVFSCSVMHEALHNHYTQKSLSLSPGK

SEQ ID NO: 249 - protein, 455 aa, Artificial sequence
  EM1 mAb HC1
QVQLVESGGGVVQPGRSLRLSCAASGFTFSTYGMHWVRQAPGKGLEWVAVIWDDGSYKYYGDSVKGRFTISRDNSKNTLYLQMNSLRAEDTAVYYCARDGITMVRGVMKDYFDYWGQGTLVTVSSASTKGPSVFPLAPSSKSTSGGTAALGCLVKDYFPEPVTVSWNSGALTSGVHTFPAVLQSSGLYSLSSVVTVPSSSLGTQTYICNVNHKPSNTKVDKRVEPKSCDKTHTCPPCPAPELLGGPSVFLFPPKPKDTLMISRTPEVTCVVVDVSHEDPEVKFNWYVDGVEVHNAKTKPREEQYNSTYRVVSVLTVLHQDWLNGKEYKCKVSNKALPAPIEKTISKAKGQPREPQVYTLPPSREEMTKNQVSLTCLVKGFYPSDIAVEWESNGQPENNYKTTPPVLDSDGSFLLYSKLTVDKSRWQQGNVFSCSVMHEALHNHYTQKSLSLSPGK

SEQ ID NO: 250 - protein, 214 aa, Artificial sequence
  EM1 mAb LC1
AIQLTQSPSSLSASVGDRVTITCRASQDISSALVWYQQKPGKAPKLLIYDASSLESGVPSRFSGSESGTDFTLTISSLQPEDFATYYCQQFNSYPLTFGGGTKVEIKRTVAAPSVFIFPPSDEQLKSGTASVVCLLNNFYPREAKVQWKVDNALQSGNSQESVTEQDSKDSTYSLSSTLTLSKADYEKHKVYACEVTHQGLSSPVTKSFNRGEC

SEQ ID NO: 251 - protein, 449 aa, Artificial sequence
  EM1 mAb HC2
QVQLVQSGAEVKKPGASVKVSCETSGYTFTSYGISWVRQAPGHGLEWMGWISAYNGYTNYAQKLQGRVTMTTDTSTSTAYMELRSLRSDDTAVYYCARDLRGTNYFDYWGQGTLVTVSSASTKGPSVFPLAPSSKSTSGGTAALGCLVKDYFPEPVTVSWNSGALTSGVHTFPAVLQSSGLYSLSSVVTVPSSSLGTQTYICNVNHKPSNTKVDKRVEPKSCDKTHTCPPCPAPELLGGPSVFLFPPKPKDTLMISRTPEVTCVVVDVSHEDPEVKFNWYVDGVEVHNAKTKPREEQYNSTYRVVSVLTVLHQDWLNGKEYKCKVSNKALPAPIEKTISKAKGQPREPQVYTLPPSREEMTKNQVSLTCLVKGFYPSDIAVEWESNGQPENNYKTTPPVLDSDGSFFLYSRLTVDKSRWQQGNVFSCSVMHEALHNHYTQKSLSLSPGK

SEQ ID NO: 252 - protein, 214 aa, Artificial sequence
  EM1 mAb LC2
DIQMTQSPSSVSASVGDRVTITCRASQGISNWLAWFQHKPGKAPKLLIYAASSLLSGVPSRFSGSGSGTDFTLTISSLQPEDFATYYCQQANSFPITFGQGTRLEIKRTVAAPSVFIFPPSDEQLKSGTASVVCLLNNFYPREAKVQWKVDNALQSGNSQESVTEQDSKDSTYSLSSTLTLSKADYEKHKVYACEVTHQGLSSPVTKSFNRGEC

SEQ ID NO: 253 - DNA, 1807 bp, Artificial sequence
  PTBB28 HC1 DNA
cagctgagttgttgtgttctgataagagtcagaggtaactcccgttgcggtgctgttaacggtggagggcagtgtagtctgagcagtactcgttgctgccgcgcgcgccaccagacataatagctgacagactaacagactgttcctttccatgggtcttttctgcagtcaccgtccttgacacgaagcttgccgccaccatggcttgggtgtggaccttgctattcctgatggcagctgcccaaagtatacaggcccaggtgcagctggtgcagagcggcgcggaagtgaaaaaaccgggcagcagcgtgaaagtgagctgcaaagcgagcggcggcacctttagcagctatgcgattagctgggtgcgccaggcgccgggccagggcctggaatggatgggcggcattattccgatttttgacaccgcgaactatgcgcagaaatttcagggccgcgtgaccattaccgcggatgaaagcaccagcaccgcgtatatggaactgagcagcctgcgcagcgaagataccgcggtgtattattgcgcgcgccctggtctcgctgcggcttatgatactggttccttggactattggggccagggcaccctggtgaccgtgagcagcgcctccaccaagggcccatcggtcttccccctggcgccctgctccaggagcacctccgagagcacagccgccctgggctgcctggtcaaggactacttccccgaaccggtgacggtgtcgtggaactcaggcgctctgaccagcggcgtgcacaccttcccagctgtcctacagtcctcaggactctactccctcagcagcgtggtgaccgtgccctccagcaacttcggcacccagacctacacctgcaacgtagatcacaagcccagcaacaccaaggtggacaagacagttgagcgcaaatgttgtgtcgagtgcccaccgtgcccagcaccacctgtggcaggaccgtcagtcttcctcttccccccaaaacccaaggacaccctcatgatctcccggacccctgaggtcacgtgcgtggtggtggacgtgagccacgaagaccccgaggtccagttcaactggtacgtggacggcgtggaggtgcataatgccaagacaaagccacgggaggagcagttcaacagcacgttccgtgtggtcagcgtcctcaccgttgtgcaccaggactggctgaacggcaaggagtacaagtgcaaggtctccaacaaaggcctcccagcccccatcgagaaaaccatctccaaaaccaaagggcagccccgagaaccacaggtgtacaccctgcccccatcccgggaggagatgaccaagaaccaggtcagcctgacctgcctggtcaaaggcttctaccccagcgacatcgccgtggagtgggagagcaatgggcagccggagaacaactacaagaccacacctcccatgctggactccgacggctccttcctgctctacagcaagctcaccgtggacaagagcaggtggcagcaggggaacgtcttctcatgctccgtgatgcatgaggctctgcacaaccactacacgcagaagagcctctccctgtctccgggtaaatgatagttcgaattcattgatcataatcagccataccacatttgtagaggttttacttgctttaaaaaacctcccacacctccccctgaacctgaaacataaaatgaatgcaattgttgttgttaacttgtttattgcagcttataatggttacaaataaagcaatagcatcacaaatttcacaaataaagcatttttttcac

SEQ ID NO: 254 - DNA, 1105 bp, Artificial sequence
  PTBB28 LC1 DNA
cagctgagttgttgtgttctgataagagtcagaggtaactcccgttgcggtgctgttaacggtggagggcagtgtagtctgagcagtactcgttgctgccgcgcgcgccaccagacataatagctgacagactaacagactgttcctttccatgggtcttttctgcagtcaccgtccttgacacgaagcttgccgccaccatggagacacattctcaggtctttgtatacatgttgctgtggttgtctggtgtcgagggagaaattgtgctgacccagagcccggcgaccctgagcctgagcccgggcgaacgcgcgaccctgagctgccgcgcgagccagagcgttcgctcctacctggcgtggtatcagcagaaaccgggccaggcgccgcgcctgctgatctacgacgcgagcaatcgtgcgaccggcattccggcgcgctttagcggctccggtagcggcaccgattttaccctgaccattagcagcctggaaccggaagattttgcggtgtattattgccagcaacgtaattattggccgctgacctttggccagggcaccaaagtggaaattaaacgtacggtggctgcaccatctgtcttcatcttcccgccatctgatgagcagttgaaatctggaactgcctctgttgtgtgcctgctgaataacttctatcccagagaggccaaagtacagtggaaggtggataacgccctccaatcgggtaactcccaggagagtgtcacagagcaggacagcaaggacagcacctacagcctcagcagcaccctgacgctgagcaaagcagactacgagaaacacaaagtctacgcctgcgaagtcacccatcagggcctgagctcgcccgtcacaaagagcttcaacaggggagagtgttagtgattcgaatgatcataatcagccataccacatttgtagaggttttacttgctttaaaaaacctcccacacctccccctgaacctgaaacataaaatgaatgcaattgttgttgttaacttgtttattgcagcttataatggttacaaataaagcaatagcatcacaaatttcacaaataaagcatttttttcactgcat

SEQ ID NO: 255 - DNA, 1789 bp, Artificial sequence
  PTBB28 HC2 DNA
cagctgagttgttgtgttctgataagagtcagaggtaactcccgttgcggtgctgttaacggtggagggcagtgtagtctgagcagtactcgttgctgccgcgcgcgccaccagacataatagctgacagactaacagactgttcctttccatgggtcttttctgcagtcaccgtccttgacacgaagcttgccgccaccatggcttgggtgtggaccttgctattcctgatggcagctgcccaaagtatacaggccgaagtgcagctgctggaaagcggcggcggcctggtgcagccgggcggcagcctgcgcctgagctgcgcggcaagcggctttacctttagcagctatgcgatgagctgggtgcgccaggcgccgggcaaaggcctggaatgggtgagcgcgattagcggcagcggcggcagcacctattatgcggatagcgtgaaaggccgctttaccattagccgcgataacagcaaaaacaccctgtatctgcagatgaacagcctgcgcgcggaagataccgcggtgtattattgcgcgaaatccccgtacgcgcccttggactattggggccagggcaccctggtgaccgtgagcagcgcctccaccaagggcccatcggtcttccccctggcgccctgctccaggagcacctccgagagcacagccgccctgggctgcctggtcaaggactacttccccgaaccggtgacggtgtcgtggaactcaggcgctctgaccagcggcgtgcacaccttcccagctgtcctacagtcctcaggactctactccctcagcagcgtggtgaccgtgccctccagcaacttcggcacccagacctacacctgcaacgtagatcacaagcccagcaacaccaaggtggacaagacagttgagcgcaaatgttgtgtcgagtgcccaccgtgcccagcaccacctgtggcaggaccgtcagtcttcctcttccccccaaaacccaaggacaccctcatgatctcccggacccctgaggtcacgtgcgtggtggtggacgtgagccacgaagaccccgaggtccagttcaactggtacgtggacggcgtggaggtgcataatgccaagacaaagccacgggaggagcagttcaacagcacgttccgtgtggtcagcgtcctcaccgttgtgcaccaggactggctgaacggcaaggagtacaagtgcaaggtctccaacaaaggcctcccagcccccatcgagaaaaccatctccaaaaccaaagggcagccccgagaaccacaggtgtacaccctgcccccatcccgggaggagatgaccaagaaccaggtcagcctgacctgcctggtcaaaggcttctaccccagcgacatcgccgtggagtgggagagcaatgggcagccggagaacaactacaagaccacacctcccatgctggactccgacggctccttcttcctctacagccggctcaccgtggacaagagcaggtggcagcaggggaacgtcttctcatgctccgtgatgcatgaggctctgcacaaccactacacgcagaagagcctctccctgtctccgggtaaatgatagttcgaattcattgatcataatcagccataccacatttgtagaggttttacttgctttaaaaaacctcccacacctccccctgaacctgaaacataaaatgaatgcaattgttgttgttaacttgtttattgcagcttataatggttacaaataaagcaatagcatcacaaatttcacaaataaagcatttttttcac

SEQ ID NO: 256 - DNA, 1105 bp, Artificial sequence
  PTBB28 LC2 DNA
cagctgagttgttgtgttctgataagagtcagaggtaactcccgttgcggtgctgttaacggtggagggcagtgtagtctgagcagtactcgttgctgccgcgcgcgccaccagacataatagctgacagactaacagactgttcctttccatgggtcttttctgcagtcaccgtccttgacacgaagcttgccgccaccatggagacacattctcaggtctttgtatacatgttgctgtggttgtctggtgtcgagggagaaattgtgctgacccagagcccggcgaccctgagcctgagcccgggcgaacgcgcgacccttagctgccgtgcaagtcagagtgtgaacgactacctggcgtggtatcagcagaaaccgggccaggcgccgcgcctgctgatttatgatgcgagcaaccgcgcgaccggcattccggcgcgctttagcggcagcggcagcggcaccgattttaccctgaccattagcagcctggaaccggaagattttgcggtgtattattgccagcagggtggtcacgcgccgatcacctttggccagggcaccaaagtggaaattaaacgtacggtggctgcaccatctgtcttcatcttcccgccatctgatgagcagttgaaatctggaactgcctctgttgtgtgcctgctgaataacttctatcccagagaggccaaagtacagtggaaggtggataacgccctccaatcgggtaactcccaggagagtgtcacagagcaggacagcaaggacagcacctacagcctcagcagcaccctgacgctgagcaaagcagactacgagaaacacaaagtctacgcctgcgaagtcacccatcagggcctgagctcgcccgtcacaaagagcttcaacaggggagagtgttagtgattcgaatgatcataatcagccataccacatttgtagaggttttacttgctttaaaaaacctcccacacctccccctgaacctgaaacataaaatgaatgcaattgttgttgttaacttgtttattgcagcttataatggttacaaataaagcaatagcatcacaaatttcacaaataaagcatttttttcactgcat

SEQ ID NO: 257 - DNA, 1807 bp, Artificial sequence
  PTBB30 HC1 DNA
cagctgagttgttgtgttctgataagagtcagaggtaactcccgttgcggtgctgttaacggtggagggcagtgtagtctgagcagtactcgttgctgccgcgcgcgccaccagacataatagctgacagactaacagactgttcctttccatgggtcttttctgcagtcaccgtccttgacacgaagcttgccgccaccatggcttgggtgtggaccttgctattcctgatggcagctgcccaaagtatacaggcccaggtgcagctggtgcagagcggcgcggaagtgaaaaaaccgggcagcagcgtgaaagtgagctgcaaagcgagcggcggcacctttagcagctatgcgattagctgggtgcgccaggcgccgggccagggcctggaatggatgggcggcattattccgatttttgacaccgcgaactatgcgcagaaatttcagggccgcgtgaccattaccgcggatgaaagcaccagcaccgcgtatatggaactgagcagcctgcgcagcgaagataccgcggtgtattattgcgcgcgccctggtctcgctgcggcttatgatactggttccttggactattggggccagggcaccctggtgaccgtgagcagcgcctccaccaagggcccatcggtcttccccctggcgccctgctccaggagcacctccgagagcacagccgccctgggctgcctggtcaaggactacttccccgaaccggtgacggtgtcgtggaactcaggcgctctgaccagcggcgtgcacaccttcccagctgtcctacagtcctcaggactctactccctcagcagcgtggtgaccgtgccctccagcaacttcggcacccagacctacacctgcaacgtagatcacaagcccagcaacaccaaggtggacaagacagttgagcgcaaatgttgtgtcgagtgcccaccgtgcccagcaccacctgccgcagccagctcagtcttcctcttccccccaaaacccaaggacaccctcatgatctcccggacccctgaggtcacgtgcgtggtggtggacgtgagcgccgaagaccccgaggtccagttcaactggtacgtggacggcgtggaggtgcataatgccaagacaaagccacgggaggagcagttcaacagcacgttccgtgtggtcagcgtcctcaccgttctgcaccaggactggctgaacggcaaggagtacaagtgcaaggtctccaacaaaggcctcccatcctccatcgagaaaaccatctccaaaaccaaagggcagccccgagaaccacaggtgtacaccctgcccccatcccgggaggagatgaccaagaaccaggtcagcctgacctgcctggtcaaaggcttctaccccagcgacatcgccgtggagtgggagagcaatgggcagccggagaacaactacaagaccacacctcccatgctggactccgacggctccttcctgctctacagcaagctcaccgtggacaagagcaggtggcagcaggggaacgtcttctcatgctccgtgatgcatgaggctctgcacaaccactacacgcagaagagcctctccctgtctccgggtaaatgatagttcgaattcattgatcataatcagccataccacatttgtagaggttttacttgctttaaaaaacctcccacacctccccctgaacctgaaacataaaatgaatgcaattgttgttgttaacttgtttattgcagcttataatggttacaaataaagcaatagcatcacaaatttcacaaataaagcatttttttcac

SEQ ID NO: 258 - DNA, 1105 bp, Artificial sequence; identical to SEQ ID NO: 254
  PTBB30 LC1 DNA

SEQ ID NO: 259 - DNA, 1789 bp, Artificial sequence
  PTBB30 HC2 DNA
cagctgagttgttgtgttctgataagagtcagaggtaactcccgttgcggtgctgttaacggtggagggcagtgtagtctgagcagtactcgttgctgccgcgcgcgccaccagacataatagctgacagactaacagactgttcctttccatgggtcttttctgcagtcaccgtccttgacacgaagcttgccgccaccatggcttgggtgtggaccttgctattcctgatggcagctgcccaaagtatacaggccgaagtgcagctgctggaaagcggcggcggcctggtgcagccgggcggcagcctgcgcctgagctgcgcggcaagcggctttacctttagcagctatgcgatgagctgggtgcgccaggcgccgggcaaaggcctggaatgggtgagcgcgattagcggcagcggcggcagcacctattatgcggatagcgtgaaaggccgctttaccattagccgcgataacagcaaaaacaccctgtatctgcagatgaacagcctgcgcgcggaagataccgcggtgtattattgcgcgaaatccccgtacgcgcccttggactattggggccagggcaccctggtgaccgtgagcagcgcctccaccaagggcccatcggtcttccccctggcgccctgctccaggagcacctccgagagcacagccgccctgggctgcctggtcaaggactacttccccgaaccggtgacggtgtcgtggaactcaggcgctctgaccagcggcgtgcacaccttcccagctgtcctacagtcctcaggactctactccctcagcagcgtggtgaccgtgccctccagcaacttcggcacccagacctacacctgcaacgtagatcacaagcccagcaacaccaaggtggacaagacagttgagcgcaaatgttgtgtcgagtgcccaccgtgcccagcaccacctgccgcagccagctcagtcttcctcttccccccaaaacccaaggacaccctcatgatctcccggacccctgaggtcacgtgcgtggtggtggacgtgagcgccgaagaccccgaggtccagttcaactggtacgtggacggcgtggaggtgcataatgccaagacaaagccacgggaggagcagttcaacagcacgttccgtgtggtcagcgtcctcaccgttctgcaccaggactggctgaacggcaaggagtacaagtgcaaggtctccaacaaaggcctcccatcctccatcgagaaaaccatctccaaaaccaaagggcagccccgagaaccacaggtgtacaccctgcccccatcccgggaggagatgaccaagaaccaggtcagcctgacctgcctggtcaaaggcttctaccccagcgacatcgccgtggagtgggagagcaatgggcagccggagaacaactacaagaccacacctcccatgctggactccgacggctccttcttcctctacagccggctcaccgtggacaagagcaggtggcagcaggggaacgtcttctcatgctccgtgatgcatgaggctctgcacaaccactacacgcagaagagcctctccctgtctccgggtaaatgatagttcgaattcattgatcataatcagccataccacatttgtagaggttttacttgctttaaaaaacctcccacacctccccctgaacctgaaacataaaatgaatgcaattgttgttgttaacttgtttattgcagcttataatggttacaaataaagcaatagcatcacaaatttcacaaataaagcatttttttcac

SEQ ID NO: 260 - DNA, 1105 bp, Artificial sequence; identical to SEQ ID NO: 256
  PTBB30 LC2 DNA

SEQ ID NO: 261 - protein, 16 aa, Homo sapiens
WGKGACPVFECGNVVL

SEQ ID NO: 262 - protein, 7 aa, Homo sapiens
DERDVNY

SEQ ID NO: 263 - protein, 13 aa, Homo sapiens
RIQIPGIMNDEKF

SEQ ID NO: 264 - protein, 306 aa, Homo sapiens
APLKIQAYFNETADLPCQFANSQNQSLSELVVFWQDQENLVLNEVYLGKEKFDSVHSKYMGRTSFDSDSWTLRLHNLQIKDKGLYQCIIHHKKPTGMIRIHQMNSELSVLANFSQPEIVPISNITENVYINLTCSSIHGYPEPKKMSVLLRTKNSTIEYDGVMQKSQDNVTELYDVSISLSVSFPDVTSNMTIFCILETDKTRLLSSPFSIELEDPQPPPDHIPWITAVLPTVIICVMVFCLILWKWKKKKRPRNSYKCGTNTMEREESEQTKKREKIHIPERSDEAQRVFKSSKTSSCDKSDTCF

SEQ ID NO: 265 - protein, 254 aa, Homo sapiens
VIHVTKEVKEVATLSCGHNVSVEELAQTRIYWQKEKKMVLTMMSGDMNIWPEYKNRTIFDITNNLSIVILALRPSDEGTYECVVLKYEKDAFKREHLAEVTLSVKADFPTPSISDFEIPTSNIRRIICSTSGGFPEPHLSWLENGEELNAINTTVSQDPETELYAVSSKLDFNMTTNHSFMCLIKYGHLRVNQTFNWNTTKQEHFPDNLLPSWAITLISVNGIFVICCLTYCFAPRCRERRRNERLRRESVRPV

SEQ ID NO: 266 - protein, 202 aa, Homo sapiens
NKILVKQSPMLVAYDNAVNLSCKYSYNLFSREFRASLHKGLDSAVEVCVVYGNYSQQLQVYSKTGFNCDGKLGNESVTFYLQNLYVNQTDIYFCKIEVMYPPPYLDNEKSNGTIIHVKGKHLCPSPLFPGPSKPFWVLVVVGGVLACYSLLVTVAFIIFWVRSKRSRLLHSDYMNMTPRRPGPTRKHYQPYAPPRDFAAYRS

SEQ ID NO: 267 - protein, 179 aa, Homo sapiens
EINGSANYEMFIFHNGGVQILCKYPDIVQQFKMQLLKGGQILCDLTKTKGSGNTVSIKSLKFCHSQLSNNSVSFFLYNLDHSHANYYFCNLSIFDPPPFKVTLTGGYLHIYESQLCCQLKFWLPIGCAAFVVVCILGCILICWLTKKKYSSSVHDPNGEYMFMRAVNTAKKSRLTDVTL

SEQ ID NO: 268 - protein, 284 aa, Homo sapiens
DTQEKEVRAMVGSDVELSCACPEGSRFDLNDVYVYWQTSESKTVVTYHIPQNSSLENVDSRYRNRALMSPAGMLRGDFSLRLFNVTPQDEQKFHCLVLSQSLGFQEVLSVEVTLHVAANFSVPVVSAPHSPSQDELTFTCTSINGYPRPNVYWINKTDNSLLDQALQNDTVFLNMRGLYDVVSVLRIARTPSVNIGCCIENVLLQQNLTVGSQTGNDIGERDKITENPVSTGEKNAATWSILAVLCLLVVVAVAIGWVCRDRCLQHSYAGAWAVSPETELTGHV

SEQ ID NO: 269 - protein, 260 aa, Homo sapiens
LSVQQGPNLLQVRQGSQATLVCQVDQATAWERLRVKWTKDGAILCQPYITNGSLSLGVCGPQGRLSWQAPSHLTLQLDPVSLNHSGAYVCWAAVEIPELEEAEGNITRLFVDPDDPTQNRNRIASFPGFLFVLLGVGSMGVAAIVWGAWFWGRRSCQQRDSGNSPGNAFYSNVLYRPRGAPKKSEDCSGEGKDQRGQSIYSTSFPQPAPRQPHLASRPCPSPRPCPSPRPGHPVSMVRVSPRPSPTQQPRPKGFPKVGEE

SEQ ID NO: 270 - protein, 257 aa, Homo sapiens
EPPTACREKQYLINSQCCSLCQPGQKLVSDCTEFTETECLPCGESEFLDTWNRETHCHQHKYCDPNLGLRVQQKGTSETDTICTCEEGWHCTSEACESCVLHRSCSPGFGVKQIATGVSDTICEPCPVGFFSNVSSAFEKCHPWTSCETKDLVVQQAGTNKTDVVCGPQDRLRALVVIPIIFGILFAILLVLVFIKKVAKKPTNKAPHPKQEPQEINFPDDLPGSNTAAPVQETLHGCQPVTQEDGKESRISVQERQ

SEQ ID NO: 271 - protein, 216 aa, Homo sapiens
QRPTGGPGCGPGRLLLGTGTDARCCRVHTTRCCRDYPGEECCSEWDCMCVQPEFHCGDPCCTTCRHHPCPPGQGVQSQGKFSFGFQCIDCASGTFSGGHEGHCKPWTDCTQFGFLTVFPGNKTHNAVCVPGSPPAEPLGWLTVVLLAVAACVLLLTSAQLGLHIWQLRSQCMWPRETQLLLEVPPSTEDARSCQFPEEERGERSAEEKGRLGDLWV

SEQ ID NO: 272 - protein, 254 aa, Homo sapiens
MEYASDASLDPEAPWPPAPRARACRVLPWALVAGLLLLLLLAAACAVFLACPWAVSGARASPGSAASPRLREGPELSPDDPAGLLDLRQGMFAQLVAQNVLLIDGPLSWYSDPGLAGVSLTGGLSYKEDTKELVVAKAGVYYVFFQLELRRVVAGEGSGSVSLALHLQPLRSAAGAAALALTVDLPPASSEARNSAFGFQGRLLHLSAGQRLGVHLHTEARARHAWQLTQGATVLGLFRVTPEIPAGLPSPRSE

SEQ ID NO: 273 - protein, 183 aa, Homo sapiens
MERVQPLEENVGNAARPRFERNKLLLVASVIQGLGLLLCFTYICLHFSALQVSHRYPRIQSIKVQFTEYKKEKGFILTSQKEDEIMKVQNNSVIINCDGFYLISLKGYFSQEVNISLHYQKDEEPLFQLKKVRSVNSLMVASLTYKDKVYLNVTTDNTSLDDFHVNGGELILIHQNPGEFCVL

SEQ ID NO: 274 - protein, 155 aa, Homo sapiens
QRFAQAQQQLPLESLGWDVAELQLNHTGPQQDPRLYWQGGPALGRSFLHGPELDKGQLRIHRDGIYMVHIQVTLAICSSTTASRHHPTTLAVGICSPASRSISLLRLSFHQGCTIASQRLTPLARGDTLCTNLTGTLLPSRNTDETFFGVQWVRP

SEQ ID NO: 275 - protein, 240 aa, Homo sapiens
MIETYNQTSPRSAATGLPISMKIFMYLLTVFLITQMIGSALFAVYLHRRLDKIEDERNLHEDFVFMKTIQRCNTGERSLSLLNCEEIKSQFEGFVKDIMLNKEETKKENSFEMQKVLQWAEKGYYTMSNNLVTLENGKQLTVKRQGLYYIYAQVTFCSNREASSQAPFIASLCLKSPGRFERILLRAANTHSSAKPCGQQSIHLGGVFELQPGASVFVNVTDPSQVSHGTGFTSFGLLKL

SEQ ID NO: 276 - protein, 393 aa, Homo sapiens
QGGTRSPRCDCAGDFHKKIGLFCCRGCPAGHYLKAPCTEPCGNSTCLVCPQDTFLAWENHHNSECARCQACDEQASQVALENCSAVADTRCGCKPGWFVECQVSQCVSSSPFYCQPCLDCGALHRHTRLLCSRRDTDCGTCLPGFYEHGDGCVSCPTSTLGSCPERCAAVCGWRQMFWVQVLLAGLVVPLLLGATLTYTYRHCWPHKPLVTADEAGMEALTPPPATHLSPLDSAHTLLAPPDSSEKICTVQLVGNSWTPGYPETQEALCPQVTWSWDQLPSRALGPAAAPTLSPESPAGSPAMMLQPGPQLYDVMDAVPARRWKEFVRTLGLREAEIEAVEVEIGRFRDQQYEMLKRWRQQQPAGLGAVYAALERMGLDGCVEDLRSRLQRGP

SEQ ID NO: 277 - protein, 240 aa, Homo sapiens
MEESVVRPSVFVVDGQTDIPFTRLGRSHRRQSCSVARVGLGLLLLLMGAGLAVQGWFLLQLHWRLGEMVTRLPDGPAGSWEQLIQERRSHEVNPAAHLTGANSSLTGSGGPLLWETQLGLAFLRGLSYHDGALVVTKAGYYYIYSKVQLGGVGCPLGLASTITHGLYKRTPRYPEELELLVSQQSPCGRATSSSRVWWDSSFLGGVVHLEAGEKVVVRVLDERLVRLRDGTRSYFGAFMV

SEQ ID NO: 278 - protein, 199 aa, Homo sapiens
MTLHPSPITCEFLFSTALISPKMCLSHLENMPLSHSRTQGAQRSSWKLWLFCSIVMLLFLCSFSWLIFIFLQLETAKEPCMAKFGPLPSKWQMASSEPPCVNKVSDWKLEILQNGLYLIYGQVAPNANYNDVAPFEVRLYKNKDMIQTLTNKSKIQNVGGTYELHVGDTIDLIFNSEHQVLKNNTYWGIILLANPQFIS

SEQ ID NO: 279 - protein, 277 aa, Homo sapiens
MCVGARRLGRGPCAALLLLGLGLSTVTGLHCVGDTYPSNDRCCHECRPGNGMVSRCSRSQNTVCRPCGPGFYNDVVSSKPCKPCTWCNLRSGSERKQLCTATQDTVCRCRAGTQPLDSYKPGVDCAPCPPGHFSPGDNQACKPWTNCTLAGKHTLQPASNSSDAICEDRDPPATQPQETQGPPARPITVQPTEAWPRTSQGPSTRPVEVPGGRAVAAILGLGLVLGLLGPLAILLALYLLRRDQRLPPDAHKPPGGGSFRTPIQEEQADAHSTLAKI

SEQ ID NO: 280 - protein, 260 aa, Homo sapiens
MARPHPWWLCVLGTLVGLSATPAPKSCPERHYWAQGKLCCQMCEPGTFLVKDCDQHRKAAQCDPCIPGVSFSPDHHTRPHCESCRHCNSGLLVRNCTITANAECACRNGWQCRDKECTECDPLPNPSLTARSSQALSPHPQPTHLPYVSEMLEARTAGHMQTLADFRQLPARTLSTHWPPQRSLCSSDFIRILVIFSGMFLVFTLAGALFLHQRRKYRSNKGESPVEPAEPCHYSCPREEEGSTIPIQEDYRKPEPACSP

SEQ ID NO: 281 - protein, 255 aa, Homo sapiens
MGNSCYNIVATLLLVLNFERTRSLQDPCSNCPAGTFCDNNRNQICSPCPPNSFSSAGGQRTCDICRQCKGVFRTRKECSSTSNAECDCTPGFHCLGAGCSMCEQDCKQGQELTKKGCKDCCFGTFNDQKRGICRPWTNCSLDGKSVLVNGTKERDVVCGPSPADLSPGASSVTPPAPAREPGHSPQIISFFLALTSTALLFLLFFLTLRFSVVKRGRKKLLYIFKQPFMRPVQTTQEEDGCSCRFPEEEEGGCEL

SEQ ID NO: 282 - protein, 216 aa, Homo sapiens
MGWIRGRRSRHSWEMSEFHNYNLDLKKSDFSTRWQKQRCPVVKSKCRENASPFFFCCFIAVAMGIRFIIMVAIWSAVFLNSLFNQEVQIPLTESYCGPCPKNWICYKNNCYQFFDESKNWYESQASCMSQNASLLKVYSKEDQDLLKLVKSYHWMGLVHIPTNGSWQWEDGSILSPNLLTIIEMQKGDCALYASSFKGYIENCSTPNTYICMQRTV

SEQ ID NO: 283 - protein, 194 aa, Homo sapiens
QGHLVHMTVVSGSNVTLNISESLPENYKQLTWFYTFDQKIVEWDSRKSKYFESKFKGRVRLDPQSGALYISKVQKEDNSTYIMRVLKKTGNEQEWKIKLQVLDPVPKPVIKIEKIEDMDDNCYLKLSCVIPGESVNYTWYGDKRPFPKELQNSVLETTLMPHNYSRCYTCQVSNSVSSKNGTVCLSPPCTLARS

SEQ ID NO: 284 - protein, 318 aa, Homo sapiens
EEVLWHTSVPFAENMSLECVYPSMGILTQVEWFKIGTQQDSIAIFSPTHGMVIRKPYAERVYFLNSTMASNNMTLFFRNASEDDVGYYSCSLYTYPQGTWQKVIQVVQSDSFEAAVPSNSHIVSEPGKNVTLTCQPQMTWPVQAVRWEKIQPRQIDLLTYCNLVHGRNFTSKFPRQIVSNCSHGRWSVIVIPDVTVSDSGLYRCYLQASAGENETFVMRLTVAEGKTDNQYTLFVAGGTVLLLLFVISITTIIVIFLNRRRRRERRDLFTESWDTQKAPNNYRSPISTSQPTNQSMDDTREDIYVNYPTFSRRPKTRV

SEQ ID NO: 285 - protein, 360 aa, Homo sapiens
EPHSLRYNLTVLSWDGSVQSGFLTEVHLDGQPFLRCDRQKCRAKPQGQWAEDVLGNKTWDRETRDLTGNGKDLRMTLAHIKDQKEGLHSLQEIRVCEIHEDNSTRSSQHFYYDGELFLSQNLETKEWTMPQSSRAQTLAMNVRNFLKEDAMKTKTHYHAMHADCLQELRRYLKSGVVLRRTVPPMVNVTRSEASEGNITVTCRASGFYPWNITLSWRQDGVSLSHDTQQWGDVLPDGNGTYQTWVATRICQGEEQRFTCYMEHSGNHSTHPVPSGKVLVLQSHWQTFHVSAVAAAAIFVIIIFYVRCCKKKTSAAEGPELVSLQVLDQHPVGTSDHRDATQLGFQPLMSDLGSTGSTEGA

SEQ ID NO: 286 - protein, 279 aa, Homo sapiens
FKVATPYSLYVCPEGQNVTLTCRLLGPVDKGHDVTFYKTWYRSSRGEVQTCSERRPIRNLTFQDLHLHHGGHQAANTSHDLAQRHGLESASDHHGNFSITMRNLTLLDSGLYCCLVVEIRHHHSEHRVHGAMELQVQTGKDAPSNCVVYPSSSQDSENITAAALATGACIVGILCLPLILLLVYKQRQAASNRRAQELVRMDSNIQGIENPGFEASPPAQGIPEAKVRHPLSYVAQRQPSESGRHLLSEPSTPLSPPGPGDVFFPSLDPVPDSPNFEVI

SEQ ID NO: 287 - protein, 432 aa, Homo sapiens
KQSEDFRVIGPAHPILAGVGEDALLTCQLLPKRTTMHVEVRWYRSEPSTPVFVHRDGVEVTEMQMEEYRGWVEWIENGIAKGNVALKIHNIQPSDNGQYWCHFQDGNYCGETSLLLKVAGLGSAPSIHMEGPGESGVQLVCTARGWFPEPQVYWEDIRGEKLLAVSEHRIQDKDGLFYAEATLVVRNASAESVSCLVHNPVLTEEKGSVISLPEKLQTELASLKVNGPSQPILVRVGEDIQLTCYLSPKANAQSMEVRWDRSHRYPAVHVYMDGDHVAGEQMAEYRGRTVLVSDAIDEGRLTLQILSARPSDDGQYRCLFEKDDVYQEASLDLKVVSLGSSPLITVEGQEDGEMQPMCSSDGWFPQPHVPWRDMEGKTIPSSSQALTQGSHGLFHVQTLLRVTNISAVDVTCSISIPFLGEEKIATFSLSGW

SEQ ID NO: 288 - protein, 506 aa, Homo sapiens
LEVQVPEDPVVALVGTDATLCCSFSPEPGFSLAQLNLIWQLTDTKQLVHSFAEGQDQGSAYANRTALFPDLLAQGNASLRLQRVRVADEGSFTCFVSIRDFGSAAVSLQVAAPYSKPSMTLEPNKDLRPGDTVTITCSSYQGYPEAEVFWQDGQGVPLTGNVTTSQMANEQGLFDVHSILRVVLGANGTYSCLVRNPVLQQDAHSSVTITPQRSPTGAVEVQVPEDPVVALVGTDATLRCSFSPEPGFSLAQLNLIWQLTDTKQLVHSFTEGRDQGSAYANRTALFPDLLAQGNASLRLQRVRVADEGSFTCFVSIRDFGSAAVSLQVAAPYSKPSMTLEPNKDLRPGDTVTITCSSYRGYPEAEVFWQDGQGVPLTGNVTTSQMANEQGLFDVHSVLRVVLGANGTYSCLVRNPVLQQDAHGSVTITGQPMTFPPEALWVTVGLSVCLIALLVALAFVCWRKIKQSCEEENAGAEDQDGEGEGSKTALQPLKHSDSKEDDGQEIA

SEQ ID NO: 289 - protein, 258 aa, Homo sapiens
LIIGFGISGRHSITVTTVASAGNIGEDGILSCTFEPDIKLSDIVIQWLKEGVLGLVHEFKEGKDELSEQDEMFRGRTAVFADQVIVGNASLRLKNVQLTDAGTYKCYIITSKGKGNANLEYKTGAFSMPEVNVDYNASSETLRCEAPRWFPQPTVVWASQVDQGANFSEVSNTSFELNSENVTMKVVSVLYNVTINNTYSCMIENDIAKATGDIKVTESEIKRRSHLQLLNSKASLCVSSFFAISWALLPLSPYLMLK

SEQ ID NO: 290 - protein, 245 aa, Homo sapiens
LPSCKEDEYPVGSECCPKCSPGYRVKEACGELTGTVCEPCPPGTYIAHLNGLSKCLQCQMCDPAMGLRASRNCSRTENAVCGCSPGHFCIVQDGDHCAACRAYATSSPGQRVQKGGTESQDTLCQNCPPGTFSPNGTLEECQHQTKCSWLVTKAGAGTSSSHWVWWFLSGSLVIVIVCSTVGLIICVKRRKPRGDVVKVIVSVQRKRQEAEGEATVIEALQAPPDVTTVAVEETIPSFTGRSPNH

SEQ ID NO: 291 - protein, 392 aa, Homo sapiens
IFPLAFFIYVPMNEQIVIGRLDEDIILPSSFERGSEVVIHWKYQDSYKVHSYYKGSDHLESQDPRYANRTSLFYNEIQNGNASLFFRRVSLLDEGIYTCYVGTAIQVITNKVVLKVGVFLTPVMKYEKRNTNSFLICSVLSVYPRPIITWKMDNTPISENNMEETGSLDSFSINSPLNITGSNSSYECTIENSLLKQTWTGRWTMKDGLHKMQSEHVSLSCQPVNDYFSPNQDFKVTWSRMKSGTFSVLAYYLSSSQNTIINESRFSWNKELINQSDFSMNLMDLNLSDSGEYLCNISSDEYTLLTIHTVHVEPSQETASHNKGLWILVPSAILAAFLLIWSVKCCRAQLEARRSRHPADGAQQERCCVPPGERCPSAPDNGEENVPLSGKV

SEQ ID NO: 292 - protein, 188 aa, Homo sapiens
KAMHVAQPAVVLASSRGIASFVCEYASPGKATEVRVTVLRQADSQVTEVCAATYMMGNELTFLDDSICTGTSSGNQVNLTIQGLRAMDTGLYICKVELMYPPPYYLGIGNGTQIYVIDPEPCPDSDFLLWILAAVSSGLFFYSFLLTAVSLSKMLKKRSPLTTGVYVKMPPTEPECEKQFQPYFIPIN

SEQ ID NO: 293 - protein, 497 aa, Homo sapiens
VPVVWAQEGAPAQLPCSPTIPLQDLSLLRRAGVTWQHQPDSGPPAAAPGHPLAPGPHPAAPSSWGPRPRRYTVLSVGPGGLRSGRLPLQPRVQLDERGRQRGDFSLWLRPARRADAGEYRAAVHLRDRALSCRLRLRLGQASMTASPPGSLRASDWVILNCSFSRPDRPASVHWFRNRGQGRVPVRESPHHHLAESFLFLPQVSPMDSGPWGCILTYRDGFNVSIMYNLTVLGLEPPTPLTVYAGAGSRVGLPCRLPAGVGTRSFLTAKWTPPGGGPDLLVTGDNGDFTLRLEDVSQAQAGTYTCHIHLQEQQLNATVTLAIITVTPKSFGSPGSLGKLLCEVTPVSGQERFVWSSLDTPSQRSFSGPWLEAQEAQLLSQPWQCQLYQGERLLGAAVYFTELSSPGAQRSGRAPGALPAGHLLLFLILGVLSLLLLVTGAFGFHLWRRQWRPRRFSALEQGIHPPQAQSKIEELEQEPEPEPEPEPEPEPEPEPEQL

SEQ ID NO: 294 - protein, 259 aa, Homo sapiens
KESCDVQLYIKRQSEHSILAGDPFELECPVKYCANRPHVTWCKLNGTTCVKLEDRQTSWKEEKNISFFILHFEPVLPNDNGSYRCSANFQSNLIESHSTTLYVTDVKSASERPSKDEMASRPWLLYRLLPLGGLPLLITTCFCLFCCLRRHQGKQNELSDTAGREINLVDAHLKSEQTEASTRQNSQVLLSETGIYDNDPDLCFRMQEGSEVYSNPCLEENKPGIVYASLNHSVIGPNSRLARNVKEAPTEYASICVRS

SEQ ID NO: 295 - protein, 133 aa, Homo sapiens
INITSSASQEGTRLNLICTVWHKKEEAEGFVVFLCKDRSGDCSPETSLKQLRLKRDPGIDGVGEISSQLMFTISQVTPLHSGTYQCCARSQKSGIRLQGHFFSILFTETGNYTVTGLKQRQHLEFSHNEGTLS

SEQ ID NO: 296 - protein, 492 aa, Homo sapiens
QLTTESMPFNVAEGKEVLLLVHNLPQQLFGYSWYKGERVDGNRQIVGYAIGTQQATPGPANSGRETIYPNASLLIQNVTQNDTGFYTLQVIKSDLVNEEATGQFHVYPELPKPSISSNNSNPVEDKDAVAFTCEPETQDTTYLWWINNQSLPVSPRLQLSNGNRTLTLLSVTRNDTGPYECEIQNPVSANRSDPVTLNVTYGPDTPTISPSDTYYRPGANLSLSCYAASNPPAQYSWLINGTFQQSTQELFIPNITVNNSGSYTCHANNSVTGCNRTTVKTIIVTELSPVVAKPQIKASKTTVTGDKDSVNLTCSTNDTGISIRWFFKNQSLPSSERMKLSQGNTTLSINPVKREDAGTYWCEVFNPISKNQSDPIMLNVNYNALPQENGLSPGAIAGIVIGVVALVALIAVALACFLHFGKTGRASDQRDLTEHKPSVSNHTQDHSNDPPNKMNEVTYSTLNFEAQQPTQPTSASPSLTATEIIYSEVKKQ

SEQ ID NO: 297 - protein, 266 aa, Homo sapiens
QEEDLPRPSISAEPGTVIPLGSHVTFVCRGPVGVQTFRLERESRSTYNDTEDVSQASPSESEARFRIDSVSEGNAGPYRCIYYKPPKWSEQSDYLELLVKETSGGPDSPDTEPGSSAGPTQRPSDNSHNEHAPASQGLKAEHLYILIGVSVVFLFCLLLLVLFCLHRQNQIKQGPPRSKDEEQKPQQRPDLAVDVLERTADKATVNGLPEKDRETDTSALAAGSSQEVTYAQLDHWALTQRTARAVSPQSTKPMAESITYAAVARH

SEQ ID NO: 298 - protein, 390 aa, Homo sapiens
MPPSGLRLLLLLLPLLWLLVLTPGRPAAGLSTCKTIDMELVKRKRIEAIRGQILSKLRLASPPSQGEVPPGPLPEAVLALYNSTRDRVAGESAEPEPEPEADYYAKEVTRVLMVETHNEIYDKFKQSTHSIYMFFNTSELREAVPEPVLLSRAELRLLRLKLKVEQHVELYQKYSNNSWRYLSNRLLAPSDSPEWLSFDVTGVVRQWLSRGGEIEGFRLSAHCSCDSRDNTLQVDINGFTTGRRGDLATIHGMNRPFLLLMATPLERAQHLQSSRHRRALDTNYCFSSTEKNCCVRQLYIDFRKDLGWKWIHEPKGYHANFCLGPCPYIWSLDTQYSKVLALYNQHNPGASAAPCCVPQALEPLPIVYYVGRKPKVEQLSNMIVRSCKCS

SEQ ID NO: 299 - protein, 160 aa, Homo sapiens
SPGQGTQSENSCTHFPGNLPNMLRDLRDAFSRVKTFFQMKDQLDNLLLKESLLEDFKGYLGCQALSEMIQFYLEEVMPQAENQDPDIKAHVNSLGENLKTLRLRLRRCHRFLPCENKSKAVEQVKNAFNKLQEKGIYKAMSEFDIFINYIEAYMTMKIRN

SEQ ID NO: 300 - protein, 564 aa, Homo sapiens
VWEKTVNTEENVYATLGSDVNLTCQTQTVGFFVQMQWSKVTNKIDLIAVYHPQYGFYCAYGRPCESLVTFTETPENGSKWTLHLRNMSCSVSGRYECMLVLYPEGIQTKIYNLLIQTHVTADEWNSNHTIEIEINQTLEIPCFQNSSSKISSEFTYAWSVENSSTDSWVLLSKGIKEDNGTQETLISQNHLISNSTLLKDRVKLGTDYRLHLSPVQIFDDGRKFSCHIRVGPNKILRSSTTVKVFAKPEIPVIVENNSTDVLVERRFTCLLKNVFPKANITWFIDGSFLHDEKEGIYITNEERKGKDGFLELKSVLTRVHSNKPAQSDNLTIWCMALSPVPGNKVWNISSEKITFLLGSEISSTDPPLSVTESTLDTQPSPASSVSPARYPATSSVTLVDVSALRPNTTPQPSNSSMTTRGFNYPWTSSGTDTKKSVSRIPSETYSSSPSGAGSTLHDNVFTSTARAFSEVPTTANGSTKTNHVHITGIVVNKPKDGMSWPVIVAALLFCCMILFGLGVRKWCQYQKEIMERPPPFKPPPPPIKYTCIQEPNESDLPYHEMETL

SEQ ID NO: 301 - protein, 223 aa, Homo sapiens [sequence omitted]

SEQ ID NO: 302 - protein, 233 aa, Homo sapiens
MDNQGVIYSDLNLPPNPKRQQRKPKGNKNSILATEQEITYAELNLQKASQDFQGNDKTYHCKDLPSAPEKLIVGILGIICLILMASVVTIVVIPSTLIQRHNNSSLNTRTQKARHCGHCPEEWITYSNSCYYIGKERRTWEESLLACTSKNSSLLSIDNEEEMKFLSIISPSSWIGVFRNSSHHPWVTMNGLAFKHEIKDSDNAELNCAVLQVNRLKSAQCGSSIIYHCKHKL

SEQ ID NO: 303 - protein, 507 aa, Homo sapiens
QDVRVQVLPEVRGQLGGTVELPCHLLPPVPGLYISLVTWQRPDAPANHQNVAAFHPKMGPSFPSPKPGSERLSFVSAKQSTGQDTEAELQDATLALHGLTVEDEGNYTCEFATFPKGSVRGMTWLRVIAKPKNQAEAQKVTFSQDPTTVALCISKEGRPPARISWLSSLDWEAKETQVSGTLAGTVTVTSRFTLVPSGRADGVTVTCKVEHESFEEPALIPVTLSVRYPPEVSISGYDDNWYLGRTDATLSCDVRSNPEPTGYDWSTTSGTFPTSAVAQGSQLVIHAVDSLFNTTFVCTVTNAVGMGRAEQVIFVRETPNTAGAGATGGIIGGIIAAIIATAVAATGILICRQQRKEQTLQGAEEDEDLEGPPSYKPPTPKAKLEAQEMPSQLFTLGASEHSPLKTPYFDAGASCTEQEMPRYHELPTLEERSGPLHPGATSLGSPIPVPPGPPAVEDVSLDLEDEEGEEEEEYLDKINPIYDALSYSSPSDSYQGKGFVMSRAMYV

SEQ ID NO: 304 - protein, 305 aa, Homo sapiens
QLLFNKTKSVEFTFCNDTVVIPCFVTNMEAQNTTEVYVKWKFKGRDIYTFDGALNKSTVPTDFSSAKIEVSQLLKGDASLKMDKSDAVSHTGNYTCEVTELTREGETIIELKYRVVSWFSPNENILIVIFPIFAILLFWGQFGIKTLKYRSGGMDEKTIALLVAGLVITVIVIVGAILFVPGEYSLKNATGLGLIVTSTGILILLHYYVFSTAIGLTSFVIAILVIQVIAYILAVVGLSLCIAACIPMHGPLLISGLSILALAQLLGLVYMKFVASNQKTIQPPRKAVEEPLNAFKESKGMMNDE

SEQ ID NO: 305 - protein, 474 aa, Homo sapiens
EEELQVIQPDKSVLVAAGETATLRCTATSLIPVGPIQWFRGAGPGRELIYNQKEGHFPRVTTVSDLTKRNNMDFSIRIGNITPADAGTYYCVKFRKGSPDDVEFKSGAGTELSVRAKPSAPVVSGPAARATPQHTVSFTCESHGFSPRDITLKWFKNGNELSDFQTNVDPVGESVSYSIHSTAKVVLTREDVHSQVICEVAHVTLQGDPLRGTANLSETIRVPPTLEVTQQPVRAENQVNVTCQVRKFYPQRLQLTWLENGNVSRTETASTVTENKDGTYNWMSWLLVNVSAHRDDVKLTCQVEHDGQPAVSKSHDLKVSAHPKEQGSNTAAENTGSNERNIYIVVGVVCTLLVALLMAALYLVRIRQKKAQGSTSSTRLHEPEKNAREITQDTNDITYADLNLPKGKKPAPQAAEPNNHTEYASIQTSPQPASEDTLTYADLDMVHLNRTPKQPAPKPEPSFSEYASVQVPRK

SEQ ID NO: 306 - protein, 349 aa, Homo sapiens
CQGSADHVVSISGVPLQLQPNSIQTKVDSIAWKKLLPSQNGFHHILKWENGSLPSNTSNDRFSFIVKNLSLLIKAAQQQDSGLYCLEVTSISGKVQTATFQVFVFESLLPDKVEKPRLQGQGKILDRGRCQVALSCLVSRDGNVSYAWYRGSKLIQTAGNLTYLDEEVDINGTHTYTCNVSNPVSWESHTLNLTQDCQNAHQEFRFWPFLVIIVILSALFLGTLACFCVWRRKRKEKQSETSPKEFLTIYEDVKDLKTRRNHEQEQTFPGGGSTIYSMIQSQSSAPTSQEPAYTLYSLIQPSRKSGSRKRNHSPSFNSTIYEVIGKSQPKAQNPARLSRKELENFDVYS

SEQ ID NO: 307 - protein, 651 aa, Homo sapiens
KLTIESTPFNVAEGKEVLLLVHNLPQHLFGYSWYKGERVDGNRQIIGYVIGTQQATPGPAYSGREIIYPNASLLIQNIIQNDTGFYTLHVIKSDLVNEEATGQFRVYPELPKPSISSNNSKPVEDKDAVAFTCEPETQDATYLWWVNNQSLPVSPRLQLSNGNRTLTLFNVTRNDTASYKCETQNPVSARRSDSVILNVLYGPDAPTISPLNTSYRSGENLNLSCHAASNPPAQYSWFVNGTFQQSTQELFIPNITVNNSGSYTCQAHNSDTGLNRTTVTTITVYAEPPKPFITSNNSNPVEDEDAVALTCEPEIQNTTYLWWVNNQSLPVSPRLQLSNDNRTLTLLSVTRNDVGPYECGIQNKLSVDHSDPVILNVLYGPDDPTISPSYTYYRPGVNLSLSCHAASNPPAQYSWLIDGNIQQHTQELFISNITEKNSGLYTCQANNSASGHSRTTVKTITVSAELPKPSISSNNSKPVEDKDAVAFTCEPEAQNTTYLWWVNGQSLPVSPRLQLSNGNRTLTLFNVTRNDARAYVCGIQNSVSANRSDPVTLDVLYGPDTPIISPPDSSYLSGANLNLSCHSASNPSPQYSWRINGIPQQHTQVLFIAKITPNNNGTYACFVSNLATGRNNSIVKSITVSASGTSPGLSA

SEQ ID NO: 308 - protein, 355 aa, Homo sapiens
MAFSGSQAPYLSPAVPFSGTIQGGLQDGLQITVNGTVLSSSGTRFAVNFQTGFSGNDIAFHFNPRFEDGGYVVCNTRQNGSWGPEERKTHMPFQKGMPFDLCFLVQSSDFKVMVNGILFVQYFHRVPFHRVDTISVNGSVQLSYISFQNPRTVPVQPAFSTVPFSQPVCFPPRPRGRRQKPPGVWPANPAPITQTVIHTVQSAPGQMFSTPAIPPMMYPHPAYPMPFITTILGGLYPSKSILLSGTVLPSAQRFHINLCSGNHIAFHLNPRFDENAVVRNTQIDNSWGSEERSLPRKMPFVRGQSFSVWILCEAHCLKVAVDGQHLFEYYHRLRNLPTINRLEVGGDIQLTHVQT

SEQ ID NO: 309 - protein, 119 aa, Artificial sequence
  OX40 antiboyd VH
QVQLVQSGAEVKKPGASVKVSCKASGYTFTSYVMHWVRQAPGQRLEWIGYINPYNDGTKYNEKFKGRATLTSDKSASTAYMELSSLRSEDTAVYYCANYYGSSLSMDYWGQGTLVTVSS

SEQ ID NO: 310 - protein, 107 aa, Artificial sequence
  OX40 antibody VL
DIQMTQSPSSLSASVGDRVTITCRASQDISNYLNWYQQKPGKAVKLLIYYTSRLHSGVPSRFSGSGSGTDYTLTISSLQPEDFATYFCQQGNTLPWTFGQGTKVEIK

SEQ ID NO: 311 - protein, 121 aa, Artificial sequence
  OX40 antibody VH
QVQLVQSGAEVKKPGSSVKVSCKASGYTFKDYTMHWVRQAPGQGLEWMGGIYPNNGGSTYNQNFKDRVTITADKSTSTAYMELSSLRSEDTAVYYCARMGYHGPHLDFDVWGQGTTVTVSS

SEQ ID NO: 312 - protein, 107 aa, Artificial sequence
  OX40 antibody VL
DIQMTQSPSSLSASVGDRVTITCKASQDVGAAVAWYQQKPGKAPKLLIYWASTRHTGVPSRFSGSGSGTDFTLTISSLQPEDFATYYCQQYINYPLTFGGGTKVEIK